European Patent Specification EP 3 472 318 B1, published September 6, 2023. Title: METHODS AND COMPOSITIONS FOR TRANSDUCING LYMPOHOCYTES AND REGULATING THE ACTIVITY THEREOF. Applicant: F1 Oncology, Inc. The sequence listing filed with the application follows.

SEQUENCE LISTING (291 sequences)

SEQ ID NO: 1 - protein, 42 aa, Homo sapiens
KRGRKKLLYIFKQPFMRPVQTTQEEDGCSCRFPEEEEGGCEL

SEQ ID NO: 2 - protein, 41 aa, Homo sapiens
RSKRSRLLHSDYMNMTPRRPGPTRKHYQPYAPPRDFAAYRS

SEQ ID NO: 3 - protein, 41 aa, Homo sapiens
RSKRSRLLHSDYMNMTPRRPGPTRKHYQAYAAARDFAAYRS

SEQ ID NO: 4 - protein, 35 aa, Homo sapiens
TKKKYSSSVHDPNGEYMFMRAVNTAKKSRLTDVTL

SEQ ID NO: 5 - protein, 37 aa, Homo sapiens
RRDQRLPPDAHKPPGGGSFRTPIQEEQADAHSTLAKI

SEQ ID NO: 6 - protein, 49 aa, Homo sapiens
HQRRKYRSNKGESPVEPAEPCRYSCPREEEGSTIPIQEDYRKPEPACSP

SEQ ID NO: 7 - protein, 114 aa, Homo sapiens
CCLRRHQGKQNELSDTAGREINLVDAHLKSEQTEASTRQNSQVLLSETGIYDNDPDLCFRMQEGSEVYSNPCLEENKPGIVYASLNHSVIGPNSRLARNVKEAPTEYASICVRS

SEQ ID NO: 8 - protein, 187 aa, Homo sapiens
RRACRKRIRQKLHLCYPVQTSQPKLELVDSRPRRSSTQLRSGASVTEPVAEERGLMSQPLMETCHSVGAAYLESLPLQDASPAGGPSSPRDLPEPRVSTEHTNNKIEKIYIMKADTVIVGTVKAELPEGRGLAGPAEPELEEELEADHTPHYPEQETEPPLGSCSDVMLSVEEEGKEDPLPTAASGK

SEQ ID NO: 9 - protein, 54 aa, Homo sapiens
HIWQLRSQCMWPRETQLLLEVPPSTEDARSCQFPEEERGERSAEEKGRLGDLWV

SEQ ID NO: 10 - protein, 60 aa, Homo sapiens
CVKRRKPRGDVVKVIVSVQRKRQEAEGEATVIEALQAPPDVTTVAVEETIPSFTGRSPNH

SEQ ID NO: 11 - protein, 163 aa, Homo sapiens
MKWKALFTAAILQAQLPITEAQSFGLLDPKLCYLLDGILFIYGVILTALFLRVKFSRSADAPAYQQGQNQLYNELNLGRREEYDVLDKRRGRDPEMGGKPRRKNPQEGLYNELQKDKMAEAYSEIGMKGERRRGKGHDGLYQGLSTATKDTYDALHMQALPPR

SEQ ID NO: 12 - protein, 164 aa, Homo sapiens
MKWKALFTAAILQAQLPITEAQSFGLLDPKLCYLLDGILFIYGVILTALFLRVKFSRSADAPAYQQGQNQLYNELNLGRREEYDVLDKRRGRDPEMGGKPQRRKNPQEGLYNELQKDKMAEAYSEIGMKGERRRGKGHDGLYQGLSTATKDTYDALHMQALPPR

SEQ ID NO: 13 - protein, 112 aa, Homo sapiens
RVKFSRSADAPAYQQGQNQLYNELNLGRREEYDVLDKRRGRDPEMGGKPRRKNPQEGLYNELQKDKMAEAYSEIGMKGERRRGKGHDGLYQGLSTATKDTYDALHMQALPPR

SEQ ID NO: 14 - protein, 21 aa, Homo sapiens
NQLYNELNLGRREEYDVLDKR

SEQ ID NO: 15 - protein, 22 aa, Homo sapiens
EGLYNELQKDKMAEAYSEIGMK

SEQ ID NO: 16 - protein, 21 aa, Homo sapiens
DGLYQGLSTATKDTYDALHMQ

SEQ ID NO: 17 - protein, 171 aa, Homo sapiens
MEHSTFLSGLVLATLLSQVSPFKIPIEELEDRVFVNCNTSITWVEGTVGTLLSDITRLDLGKRILDPRGIYRCNGTDIYKDKESTVQVHYRMCQSCVELDPATVAGIIVTDVIATLLLALGVFCFAGHETGRLSGAADTQALLRNDQVYQPLRDRDDAQYSHLGGNWARNK

SEQ ID NO: 18 - protein, 127 aa, Homo sapiens
MEHSTFLSGLVLATLLSQVSPFKIPIEELEDRVFVNCNTSITWVEGTVGTLLSDITRLDLGKRILDPRGIYRCNGTDIYKDKESTVQVHYRTADTQALLRNDQVYQPLRDRDDAQYSHLGGNWARNK

SEQ ID NO: 19 - protein, 21 aa, Homo sapiens
DQVYQPLRDRDDAQYSHLGGN

SEQ ID NO: 20 - protein, 206 aa, Homo sapiens
MQSGTHWRVLGLCLLSVGVWGQDGNEEMGGITQTPYKVSISGTTVILTCPQYPGSEILWQHNDKNIGGDEDDKNIGSDEDHLSLKEFSELEQSGYYVCYPRGSKPEDANFYLYLRARVCENCMEMDMSVATIVIVDICITGGLLLLVYYWSKNRKAKAKPVTRGAGAGGRQRGQNKERPPPVPNPDYEPIRKGQRDLYSGLNQRRI

SEQ ID NO: 21 - protein, 21 aa, Homo sapiens
NPDYEPIRKGQRDLYSGLNQR

SEQ ID NO: 22 - protein, 182 aa, Homo sapiens
MEQGKGLAVLILAIILLQGTLAQSIKGNHLVKVYDYQEDGSVLLTCDAEAKNITWFKDGKMIGFLTEDKKKWNLGSNAKDPRGMYQCKGSQNKSKPLQVYYRMCQNCIELNAATISGFLFAEIVSIFVLAVGVYFIAGQDGVRQSRASDKQTLLPNDQLYQPLKDREDDQYSHLQGNQLRRN

SEQ ID NO: 23 - protein, 21 aa, Homo sapiens
DQLYQPLKDREDDQYSHLQGN

SEQ ID NO: 24 - protein, 226 aa, Homo sapiens
MPGGPGVLQALPATIFLLFLLSAVYLGPGCQALWMHKVPASLMVSLGEDAHFQCPHNSSNNANVTWWRVLHGNYTWPPEFLGPGEDPNGTLIIQNVNKSHGGIYVCRVQEGNESYQQSCGTYLRVRQPPPRPFLDMGEGTKNRIITAEGIILLFCAVVPGTLLLFRKRWQNEKLGLDAGDEYEDENLYEGLNLDDCSMYEDISRGLQGTYQDVGSLNIGDVQLEKP

SEQ ID NO: 25 - protein, 188 aa, Homo sapiens
MPGGPGVLQALPATIFLLFLLSAVYLGPGCQALWMHKVPASLMVSLGEDAHFQCPHNSSNNANVTWWRVLHGNYTWPPEFLGPGEDPNEPPPRPFLDMGEGTKNRIITAEGIILLFCAVVPGTLLLFRKRWQNEKLGLDAGDEYEDENLYEGLNLDDCSMYEDISRGLQGTYQDVGSLNIGDVQLEKP

SEQ ID NO: 26 - protein, 21 aa, Homo sapiens
ENLYEGLNLDDCSMYEDISRG

SEQ ID NO: 27 - protein, 113 aa, Homo sapiens
MGGLEPCSRLLLLPLLLAVSGLRPVQAQAQSDCSCSTVSPGVLAGIVMGDLVLTVLIALAVYFLGRLVPRGRGAAEAATRKQRITETESPYQELQGQRSDVYSDLNTQRPYYK

SEQ ID NO: 28 - protein, 107 aa, Homo sapiens
MGGLEPCSRLLLLPLLLAVSGLRPVQAQAQSDCSCSTVSPGVLAGIVMGDLVLTVLIALAVYFLGRLVPRGRGAAEATRKQRITETESPYQELQGQRSDVYSDLNTQ

SEQ ID NO: 29 - protein, 102 aa, Homo sapiens
MGGLEPCSRLLLLPLLLAVSDCSCSTVSPGVLAGIVMGDLVLTVLIALAVYFLGRLVPRGRGAAEAATRKQRITETESPYQELQGQRSDVYSDLNTQRPYYK

SEQ ID NO: 30 - protein, 101 aa, Homo sapiens
MGGLEPCSRLLLLPLLLAVSDCSCSTVSPGVLAGIVMGDLVLTVLIALAVYFLGRLVPRGRGAAEATRKQRITETESPYQELQGQRSDVYSDLNTQRPYYK

SEQ ID NO: 31 - protein, 21 aa, Homo sapiens
ESPYQELQGQRSDVYSDLNTQ

SEQ ID NO: 32 - protein, 86 aa, Homo sapiens
MIPAVVLLLLLLVEQAAALGEPQLCYILDAILFLYGIVLTLLYCRLKIQVRKAAITSYEKSDGVYTGLSTRNQETYETLKHEKPPQ

SEQ ID NO: 33 - protein, 21 aa, Homo sapiens
DGVYTGLSTRNQETYETLKHE

SEQ ID NO: 34 - protein, 20 aa, Homo sapiens
RPRRSPAQDGKVYINMPGRG

SEQ ID NO: 35 - protein, 68 aa, Homo sapiens
FWVLVVVGGVLACYSLLVTVAFIIFWVRSKRSRLLHSDYMNMTPRRPGPTRKHYQPYAPPRDFAAYRS

SEQ ID NO: 36 - protein, 619 aa, Homo sapiens
MPDPAAHLPFFYGSISRAEAEEHLKLAGMADGLFLLRQCLRSLGGYVLSLVHDVRFHHFPIERQLNGTYAIAGGKAHCGPAELCEFYSRDPDGLPCNLRKPCNRPSGLEPQPGVFDCLRDAMVRDYVRQTWKLEGEALEQAIISQAPQVEKLIATTAHERMPWYHSSLTREEAERKLYSGAQTDGKFLLRPRKEQGTYALSLIYGKTVYHYLISQDKAGKYCIPEGTKFDTLWQLVEYLKLKADGLIYCLKEACPNSSASNASGAAAPTLPAHPSTLTHPQRRIDTLNSDGYTPEPARITSPDKPRPMPMDTSVYESPYSDPEELKDKKLFLKRDNLLIADIELGCGNFGSVRQGVYRMRKKQIDVAIKVLKQGTEKADTEEMMREAQIMHQLDNPYIVRLIGVCQAEALMLVMEMAGGGPLHKFLVGKREEIPVSNVAELLHQVSMGMKYLEEKNFVHRDLAARNVLLVNRHYAKISDFGLSKALGADDSYYTARSAGKWPLKWYAPECINFRKFSSRSDVWSYGVTMWEALSYGQKPYKKMKGPEVMAFIEQGKRMECPPECPPELYALMSDCWIYKWEDRPDFLTVEQRMRACYYSLASKVEGPPGSTQKAEAACA

SEQ ID NO: 37 - protein, 9 aa, Artificial sequence
  synthetic HA Epitope
YPYDVPDYA

SEQ ID NO: 38 - protein, 8 aa, Artificial sequence
  synthetic FLAG Epitope
DYKDDDDK

SEQ ID NO: 39 - protein, 10 aa, Artificial sequence
  synthetic c-myc Epitope
EQKLISEEDL

SEQ ID NO: 40 - protein, 5 aa, Artificial sequence
  synthetic His5 Affinity
HHHHH

SEQ ID NO: 41 - protein, 6 aa, Artificial sequence
  synthetic HisX6 Affinity
HHHHHH

SEQ ID NO: 42 - protein, 8 aa, Artificial sequence
  synthetic Strep Tag Affinity
WSHPQFEK

SEQ ID NO: 43 - protein, 5 aa, Artificial sequence
  synthetic HisX6 Affinity
RYIRS

SEQ ID NO: 44 - protein, 4 aa, Artificial sequence
  synthetic Affinity
FHHT

SEQ ID NO: 45 - protein, 17 aa, Artificial sequence
  synthetic Affinity
WEAAAREACCRECCARA

SEQ ID NO: 46 - protein, 24 aa, Homo sapiens
IYIWAPLAGTCGVLLLSLVITLYC

SEQ ID NO: 47 - protein, 23 aa, Homo sapiens
LGLLVAGVLVLLVSLGVAIHLCC

SEQ ID NO: 48 - protein, 25 aa, Homo sapiens
ALIVLGGVAGLLLFIGLGIFFCVRC

SEQ ID NO: 49 - protein, 23 aa, Homo sapiens
LCYLLDGILFIYGVILTALFLRV

SEQ ID NO: 50 - protein, 27 aa, Homo sapiens
FWVLVVVGGVLACYSLLVTVAFIIFWV

SEQ ID NO: 51 - protein, 26 aa, Homo sapiens
VAAILGLGLVLGLLGPLAILLALYLL

SEQ ID NO: 52 - protein, 24 aa, Homo sapiens
ALPAALAVISFLLGLGLGVACVLA

SEQ ID NO: 53 - protein, 15 aa, Artificial sequence
  synthetic Linker 1
GGGGSGGGGSGGGGS

SEQ ID NO: 54 - protein, 30 aa, Artificial sequence
  synthetic Linker 2
GGGGSGGGGSGGGGSGGGGSGGGGSGGGGS

SEQ ID NO: 55 - protein, 14 aa, Artificial sequence
  synthetic Linker 3
GGGGSGGGSGGGGS

SEQ ID NO: 56 - protein, 4 aa, Artificial sequence
  synthetic Linker 4
GGSG

SEQ ID NO: 57 - protein, 5 aa, Artificial sequence
  synthetic Linker 5
GGSGG

SEQ ID NO: 58 - protein, 5 aa, Artificial sequence
  synthetic Linker 6
GSGSG

SEQ ID NO: 59 - protein, 5 aa, Artificial sequence
  synthetic Linker 7
GSGGG

SEQ ID NO: 60 - protein, 5 aa, Artificial sequence
  synthetic Linker 8
GGGSG

SEQ ID NO: 61 - protein, 5 aa, Artificial sequence
  synthetic Linker 9
GSSSG

SEQ ID NO: 62 - protein, 4 aa, Artificial sequence
  synthetic Hinge 1
CPPC

SEQ ID NO: 63 - protein, 5 aa, Artificial sequence
  synthetic Hinge 2
DKTHT

SEQ ID NO: 64 - protein, 15 aa, Artificial sequence
  synthetic Hinge 3
CPEPKSCDTPPPCPR

SEQ ID NO: 65 - protein, 12 aa, Artificial sequence
  synthetic Hinge 4
ELKTPLGDTTHT

SEQ ID NO: 66 - protein, 10 aa, Artificial sequence
  synthetic Hinge 5
KSCDKTHTCP

SEQ ID NO: 67 - protein, 7 aa, Artificial sequence
  synthetic Hinge 6
KCCVDCP

SEQ ID NO: 68 - protein, 7 aa, Artificial sequence
  synthetic Hinge 7
KYGPPCP

SEQ ID NO: 69 - protein, 15 aa, Artificial sequence
  synthetic Hinge 8
EPKSCDKTHTCPPCP

SEQ ID NO: 70 - protein, 12 aa, Artificial sequence
  synthetic Hinge 9
ERKCCVECPPCP

SEQ ID NO: 71 - protein, 17 aa, Artificial sequence
  synthetic Hinge 10
ELKTPLGDTTHTCPRCP

SEQ ID NO: 72 - protein, 12 aa, Artificial sequence
  synthetic Hinge 11
SPNMVPHAHHAQ

SEQ ID NO: 73 - protein, 45 aa, Artificial sequence
  synthetic Hinge 12
TTTPAPRPPTPAPTIASQPLSLRPEACRPAAGGAVHTRGLDFACD

SEQ ID NO: 74 - protein, 21 aa, Homo sapiens
MALPVTALLLPLALLLHAARP

SEQ ID NO: 75 - protein, 24 aa, Homo sapiens
IYIWAPLAGTCGVLLLSLVITLYC

SEQ ID NO: 76 - protein, 27 aa, Homo sapiens
FWVLVVVGGVLACYSLLVTVAFIIFWV

SEQ ID NO: 77 - protein, 21 aa, Artificial sequence
  synthetic 2A-1 Cleavage signal
GSGEGRGSLLTCGDVEENPGP

SEQ ID NO: 78 - protein, 357 aa, Homo sapiens
MLLLVTSLLLCELPHPAFLLIPRKVCNGIGIGEFKDSLSINATNIKHFKNCTSISGDLHILPVAFRGDSFTHTPPLDPQELDILKTVKEITGFLLIQAWPENRTDLHAFENLEIIRGRTKQHGQFSLAVVSLNITSLGLRSLKEISDGDVIISGNKNLCYANTINWKKLFGTSGQKTKIISNRGENSCKATGQVCHALCSPEGCWGPEPRDCVSCRNVSRGRECVDKCNLLEGEPREFVENSECIQCHPECLPQAMNITCTGRGPDNCIQCAHYIDGPHCVKTCPAGVMGENNTLVWKYADAGHVCHLCHPNCTYGCTGPGLEGCPTNGPKIPSIATGMVGALLLLLVVALGIGLFM

SEQ ID NO: 79 - protein, 45 aa, Homo sapiens; identical to SEQ ID NO: 73

SEQ ID NO: 80 - protein, 39 aa, Homo sapiens
IEVMYPPPYLDNEKSNGTIIHVKGKHLCPSPLFPGPSKP

SEQ ID NO: 81 - protein, 113 aa, Homo sapiens
RVKFSRSADAPAYQQGQNQLYNELNLGRREEYDVLDKRRGRDPEMGGKPQRRKNPQEGLYNELQKDKMAEAYSEIGMKGERRRGKGHDGLYQGLSTATKDTYDALHMQALPPR

SEQ ID NO: 82 - protein, 463 aa, Homo sapiens
MTILGTTFGMVFSLLQVVSGESGYAQNGDLEDAELDDYSFSCYSQLEVNGSQHSLTCAFEDPDVNTTNLEFEICGALVEVKCLNFRKLQEIYFIETKKFLLIGKSNICVKVGEKSLTCKKIDLTTIVKPEAPFDLSVIYREGANDFVVTFNTSHLQKKYVKVLMHDVAYRQEKDENKWTHVNLSSTKLTLLQRKLQPAAMYEIKVRSIPDHYFKGFWSEWSPSYYFRTPEINNSSGEMDPILLPPCLTISILSFFSVALLVILACVLWKKRIKPIVWPSLPDHKKTLEHLCKKPRKNLNVSFNPESFLDCQIHRVDDIQARDEVEGFLQDTFPQQLEESEKQRLGGDVQSPNCPSEDVVVTPESFGRDSSLTCLAGNVSACDAPILSSSRSLDCRESGKNGPHVYQDLLLSLGTTNSTLPPPFSLQSGILTLNPVAQGQPILTSLGSNQEEAYVTMSSFYQNQ

SEQ ID NO: 83 - DNA, 13673 bp, Artificial sequence
  synthetic Dox-rapamycin inducible lentiviral genome with riboswitch
gatatctataacaagaaaatatatatataataagttatcacgtaagtagaacatgaaataacaatataattatcgtatgagttaaatcttaaaagtcacgtaaaagataatcatgcgtcattttgactcacgcggtcgttatagttcaaaatcagtgacacttaccgcattgacaagcacgcctcacgggagctccaagcggcgactgagatgtcctaaatgcacagcgacggattcgcgctatttagaaagagagagcaatatttcaagaatgcatgcgtcaattttacgcagactatctttctagggttaagacggatcgggagatctcccgatcccctatggtgcactctcagtacaatctgctctgatgccgcatagttaagccagtatctgctccctgcttgtgtgttggaggtcgctgagtagtgcgcgagcaaaatttaagctacaacaaggcaaggcttgaccgacaattgcatgaagaatctgcttagggttaggcgttttgcgctgcttcgcgatgtacgggccagatatacgcgttgacattgattattgactagttattaatagtaatcaattacggggtcattagttcatagcccatatatggagttccgcgttacataacttacggtaaatggcccgcctggctgaccgcccaacgacccccgcccattgacgtcaataatgacgtatgttcccatagtaacgccaatagggactttccattgacgtcaatgggtggagtatttacggtaaactgcccacttggcagtacatcaagtgtatcatatgccaagtacgccccctattgacgtcaatgacggtaaatggcccgcctggcattatgcccagtacatgaccttatgggactttcctacttggcagtacatctacgtattagtcatcgctattaccatggtgatgcggttttggcagtacatcaatgggcgtggatagcggtttgactcacggggatttccaagtctccaccccattgacgtcaatgggagtttgttttggaaccaaaatcaacgggactttccaaaatgtcgtaacaactccgccccattgacgcaaatgggcggtaggcgtgtacggtgggaggtctatataagcagagctctccctatcagtgatagagatctccctatcagtgatagagatcgtcgacgagctcgtttagtgaaccgtcagatcgcctggagacgccctcgaagccgcggtgcgggtgccagggcgtgccctgggtctctctggttagaccagatctgagcctgggagctctctggctaactagggaacccactgcttaagcctcaataaagcttgccttgagtgcttcaagtagtgtgtgcccgtctgttgtgtgactctggtaactagagatccctcagacccttttagtcagtgtggaaaatctctagcagtggcgcccgaacagggacttgaaagcgaaagggaaaccagaggagctctctcgacgcaggactcggcttgctgaagcgcgcacggcaagaggcgaggggcggcgactggtgagtacgccaaaaattttgactagcggaggctagaaggagagagatgggtgcgagagcgtcagtattaagcgggggagaattagatcgcgatgggaaaaaattcggttaaggccagggggaaagaaaaaatataaattaaaacatatagtatgggcaagcagggagctagaacgattcgcagttaatcctggcctgttagaaacatcagaaggctgtagacaaatactgggacagctacaaccatcccttcagacaggatcagaagaacttagatcattatataatacagtagcaaccctctattgtgtgcatcaaaggatagagataaaagacaccaaggaagctttagacaagatagaggaagagcaaaacaaaagtaagaccaccgcacagcaagcggccgctgatcttcagacctggaggaggagatatgagggacaattggagaagtgaattatataaatataaagtagtaaaaattgaaccattaggagtagcacccaccaaggcaaagagaagagtggtgcagagagaaaaaagagcagtgggaataggagctttgttccttgggttcttgggagcagcaggaagcactatgggcgcagcgtcaatgacgctgacggtacaggccagacaattattgtctggtatagtgcagcagcagaacaatttgctgagggctattgaggcgcaacagcatctgttgcaactcacagtctggggcatcaagcagctccaggcaagaatcctggctgtggaaagatacctaaaggatcaacagctcctggggatttggggttgctctggaaaactcatttgcaccactgctgtgccttggaatgctagttggagtaataaatctctggaacagatttggaatcacacgacctggatggagtgggacagagaaattaacaattacacaagcttaatacactccttaattgaagaatcgcaaaaccagcaagaaaagaatgaacaagaattattggaattagataaatgggcaagtttgtggaattggtttaacataacaaattggctgtggtatataaaattattcataatgatagtaggaggcttggtaggtttaagaatagtttttgctgtactttctatagtgaatagagttaggcagggatattcaccattatcgtttcagacccacctcccaaccccgaggggacccgacaggcccgaaggaatagaagaagaaggtggagagagagacagagacagatccattcgattagtgaacggatctcgacggtatcgattagactgtagcccaggaatatggcagctagattgtacacatttagaaggaaaagttatcttggtagcagttcatgtagccagtggatatatagaagcagaagtaattccagcagagacagggcaagaaacagcatacttcctcttaaaattagcaggaagatggccagtaaaaacagtacatacagacaatggcagcaatttcaccagtactacagttaaggccgcctgttggtgggcggggatcaagcaggaatttggcattccctacaatccccaaagtcaaggagtaatagaatctatgaataaagaattaaagaaaattataggacaggtaagagatcaggctgaacatcttaagacagcagtacaaatggcagtattcatccacaattttaaaagaaaaggggggattggggggtacagtgcaggggaaagaatagtagacataatagcaacagacatacaaactaaagaattacaaaaacaaattacaaaaattcaaaattttcgggtttattacagggacagcagagatccagtttggctgcattgatcacgtgaggggctctagactctagacacacaaaaaaccaacacacagatctaatgaaaataaagatcttttattgagaaacttatacagggtagcataatgggctactgaccccgccttcaaacctatttggagactataagtgaaaattatcactggttttggtagaagctggacatggtgacatatgcttcttcttgatttgatcccagggaagtaagaatgggctgaccctgagcaactgggttcaatgtcaggattccagattggagagaaaatggagggggcagcgtgctgtttgtagtcccaaggctaagcaggaggtcctggtacacatgaggcccattcttgccactctccctgcagtctagggacctggaagaggagagaataggggcgtcacatgcactgacattcccagccaggcatgtgagggatgaatctcttccaaagctttctggagtgacgactacatcctcagatgggcagttggggctctgcacatcccctccaagcctctgcttctcagattcttctagttgctgaggaaacgtatcttgcagaaaaccttccacttcatctctagcttgaatgtcatccaccctatgaatctggcagtccaggaaactttcaggattgaaactcacatttaaattttttcttggtttcttacaaagatgttccagagtcttcttatgatcggggagactgggccatacgataggcttaatcctttttttccataacacacaggccaagatgaccaacagagcgacagagaaaaaactcaaaatgctgatggtcaggcatggtggtagtaagataggatccatctcccctgagctattattgatctctggagttctgaagtaataacttggactccattcactccagaagcctttaaaatagtgatcagggatggatcgaactttaatctcatacattgctgccggttggagctttctctgcaggagtgtcagctttgtgctggataaattcacatgcgtccatttgttttcatccttttcctggcggtaagctacatcatgcattaaaacttttacatacttcttttgcaagtgtgatgtattaaatgtcaccacaaagtcattggctccttcccgatagatgacactcaggtcaaaaggagcctcaggtttaactatagtggttaggtctatttttttgcaggttagactcttttctccaaccttcacacatatattgctctttccaatcagtaagaatttctttgtctcgatgaaatatatctcttgtagtttcctgaaattcaggcactttacctccacgagggccccacatatttcaaattccagattggtggtgttgacatctgggtcctcaaaagcacatgtcagtgaatgctgcgatccattcacttccaactggctatagcatgagaatgagtagtcatccagttctgcatcttccaagtctccattttgagcatagccactttctccagaaacgacttgaagtaaagaaaaaaccatgccaaaagttgtacctagaattgtcattgggccgggattttcctccacgtccccgcatgttagtagacttcccctgccctcgccggagcgagggggcagggcctgcatgtgaagggcgtcgtaggtgtccttggtggctgtactgagaccctggtaaaggccatcgtgccccttgcccctccggcgctcgcctttcatcccaatctcactgtaggcctccgccatcttatctttctgcagttcattgtacaggccttcctgagggttcttccttctcggctttccccccatctcagggtcccggccacgtctcttgtccaaaacatcgtactcctctcttcgtcctagattgagctcgttatagagctggttctggccctgcttgtacgcgggggcgtctgcgctcctgctgaacttcactctcagttcacatcctccttcttcttcttctggaaatcggcagctacagccatcttcctcttgagtagtttgtactggtctcataaatggttgtttgaatatatacaggagtttctttctgccccgtttgcagtaaagggtgataaccagtgacaggagaaggaccccacaagtcccggccaagggcgcccagatgtagatatcacaggcgaagtccagccccctcgtgtgcactgcgccccccgccgctggccggcacgcctctgggcgcagggacaggggctgcgacgcgatggtgggcgccggtgttggtggtcgcggcgctggcgtcgtggttgaggagacggtgactgaggttccttggccccagtagtccatagcatagctaccaccgtagtaataatgtttggcacagtagtaaatggctgtgtcatcagtttgcagactgttcatttttaagaaaacttggctcttggagttgtccttgatgatggtcagtctggatttgagagctgaattatagtatgtggtttcactaccccatattactcccagccactccagaccctttcgtggaggctggcgaatccagcttacaccatagtcgggtaatgagacccctgagacagtgcatgtgacggacaggctctgtgagggcgccaccaggccaggtcctgactcctgcagtttcacctcagatccgccgccacccgacccaccaccgcccgagccaccgccacctgtgatctccagcttggtcccccctccgaacgtgtacggaagcgtattaccctgttggcgaagtaggtggcaatatcttcttgctccaggttgctaattgtcagagaataatctgttccagacccactgccactgaaccttgatgggactcctgagtgtaatcttgatgtatggtagatcaggagtttaacagttccatctggtttctgctgataccaatttaaatatttactaatgtcctgacttgccctgcaactgatggtgactctgtctcccagagaggcagacagggaggatgtagtctgtgtcatctggatgtccggcctggcggcgtggagcagcaaggccagcggcaggagcaaggcggtcactggtaaggccatggatcctctagatcacgacacctgaaatggaagaaaaaaactttgaaccactgtctgaggcttgagaatgaaccaagatccaaactcaaaaagggcaaattccaaggagaattacatcaagtgccaagctggcctaacttcagtctccacccactcagtgtggggaaactccatcgcataaaacccctccccccaacctaaagacgacgtactccaaaagctcgagaactaatcgaggtgcctggacggcgcccggtactcagtggagtcacatgaagcgacggctgaggacggaaaggcccttttcctttgtgtgggagaaacttatacagggtagcataatgggctactgaccccgccttcaaacctatttggagactataagtgaaaatgactcacccgcccgctctcccggcaccttcatcttgtcctttccctcagaaagaggctgggaggcagaggctgaggcagcggtggccgggacggttaggagaaaaggagtctctgctggttttattctgcagctacctccccaggaagtggaggactgtggggcctttgagaagcacctgccgacagggccaagaaattcgcactccccctttcggttcacaggcaggaagccctggaggtttgagggtttggggtgtgtgtatgtatctgtctgtctgaattttgctttttctctcatttgaccattgttttaatgctcctttttttaaaaaaaataattcttatctaattcctatcttgattggtaaagtccatctctaggcaaatacaagttctcgatggaaaacaataagtaatgtaaaatacagcatagcaaaactttaacctccaaatcaagcctctacttgaatccttttctgagggatgaataaggcataggcatcaggggctgttgccaatgtgcattagctgtttgcagcctcaccttctttcatggagtttaagatatagtgtattttcccaaggtttgaactagctcttcatttctttatgttttaaatgcactgacctcccacattccctttttagtaaaatattcagaaataatttaaatacatcattgcaatgaaaataaatgttttttattaggcagaatccagatgctcaaggcccttcataatatcccccagtttagtagttggacttagggaacaaaggaacctttaatagaaattggacagcaagaaagcgagcttagtgatacttgtgatcctctagatcacgacacctgaaatggaagaaaaaaactgcaccttcatcttgtcctttccctcagaaagaggctgggaggcagaggctgaggcagcggtggccgggacggttaggagaaaaggagtctctgctggttttattctgcagctacctccccaggaagtggaggactgtggggcctttgagaagcacctgccgacagggccaagaaattcgcactccccctttcggttcacaggcaggaagccctggaggtttgagggtttggggtgtgtgtatgtatctgtctgtctgaattttgctttttctctcatttgaccattgttttaatgctcctttttttaaaaaaaataattcttatctaattcctatcttgattggtaaagtccatctctaggcaaatacaagttctcgatggaaaacaataagtaatgtaaaatacagcatagcaaaactttaacctccaaatcaagcctctacttgaatccttttctgagggatgaataaggcataggcatcaggggctgttgccaatgtgcattagctgtttgcagcctcaccttctttcatggagtttaagatatagtgtattttcccaaggtttgaactagctcttcatttctttatgttttaaatgcactgacctcccacattccctttttagtaaaatattcagaaataatttaaatacatcattgcaatgaaaataaatgttttttattaggcagaatccagatgctcaaggcccttcataatatcccccagtttagtagttggacttagggaacaaaggaacctttaatagaaattggacagcaagaaagcgagcttagtgatacttgtaaaaagagacgcgtctctaaaagtcctttccatggctgctcgcctgtgttgccacctggattctgcgcgggacgtccttctgctacgtcccttcggccctcaatccagcggaccttccttcccgcggcctgctgccggctctgcggcctcttccgcgtcttcgccttcgccctcagacgagtcggatctccctttgggccgcctccccgcctggaattcgagctcggtacctttaagaccaatgacttacaaggcagctgtagatcttagccactttttaaaagaaaaggggggactggaagggctaattcactcccaacgaagacaagatctgctttttgcttgtactgggtctctctggttagaccagatctgagcctgggagctctctggctaactagggaacccactgcttaagcctcaataaagcttgccttgagtgcttcaagtagtgtgtgcccgtctgttgtgtgactctggtaactagagatccctcagacccttttagtcagtgtggaaaatctctagcagtagtagttcatgtcatcttattattcagtatttataacttgcaaagaaatgaatatcagagagtgagaggaacttgtttattgcagcttataatggttacaaataaagcaatagcatcacaaatttcacaaataaagcatttttttcactgcattctagttgtggtttgtccaaactcatcaatgtatcttatcatgtctggctctagctatcccgcccctaactccgcccatcccgcccctaactccgcccagttccgcccattctccgccccatggctgactaattttttttatttatgcagaggccgaggccgcctcggcctctgagctattccagaagtagtgaggaggcttttttggaggcctagggacgtatggccacaacctgggctccccgggcgcgtactccacctcacccatcatccacgctgttttatgagtaaaggagaagaacttttcactggagttgtcccaattcttgttgaattagatggtgatgttaatgggcacaaattttctgtcagtggagagggtgaaggtgatgcaacatacggaaaacttacccttaaatttatttgcactactggaaaactacctgttccatggccaacacttgtcactactttctcttatggtgttcaatgcttttcaagatacccagatcatatgaaacggcatgactttttcaagagtgccatgcccgaaggttatgtacaggaaagaactatatttttcaaagatgacgggaactacaagacacgtgctgaagtcaagtttgaaggtgatacccttgttaatagaatcgagttaaaaggtattgattttaaagaagatggaaacattcttggacacaaattggaatacaactataactcacacaatgtatacatcatggcagacaaacaaaagaatggaatcaaagttaacttcaaaattagacacaacattgaagatggaagcgttcaactagcagaccattatcaacaaaatactccaattggcgatggccctgtccttttaccagacaaccattacctgtccacacaatctgccctttcgaaagatcccaacgaaaagagagaccacatggtccttcttgagtttgtaacagctgctgggattacacatggcatggatgaactatacaaataggacctccatagaagacaccgggaccgatccaataacttcgtatagcatacattatacgaagttatgcctccggactctagcgtttaaacttaagcttgggaagttcctattccgaagttcctattctctagaaagtataggaacttctaccgagctcggatccactagtccagtgtggtggaattctgcagatatccagcacagtggcggccgctcgagtctagagggcccgtttaaacccgctgatcagcctcgactgtgccttctagttgccagccatctgttgtttgcccctcccccgtgccttccttgaccctggaaggtgccactcccactgtcctttcctaataaaatgaggaaattgcatcgcattgtctgagtaggtgtcattctattctggggggtggggtggggcaggacagcaagggggaggattgggaagacaatagcaggcatgctggggatgcggtgggctctatggcttctgaggcggaaagttaaccctagaaagataatcatattgtgacgtacgttaaagataatcatgcgtaaaattgacgcatgtgttttatcggtctgtatatcgaggtttatttattaatttgaatagatattaagttttattatatttacacttacatactaataataaattcaacaaacaatttatttatgtttatttatttattaaaaaaaaacaaaaactcaaaatttcttctataaagtaacaaaaaccagctggggctcgaagttcctatactttctagagaataggaacttctatagtgagtcgaataagggcgacacaaaatttattctaaatgcataataaatactgataacatcttatagtttgtattatattttgtattatcgttgacatgtataattttgatatcaaaaactgattttccctttattattttcgagatttattttcttaattctctttaacaaactagaaatattgtatatacaaaaaatcataaataatagatgaatagtttaattataggtgttcatcaatcgaaaaagcaacgtatcttatttaaagtgcgttgcttttttctcatttataaggttaaataattctcatatatcaagcaaagtgacaggcgcccttaaatattctgacaaatgctctttccctaaactccccccataaaaaaacccgccgaagcgggtttttacgttatttgcggattaacgattactcgttatcagaaccgcccagggggcccgagcttaagactggccgtcgttttacaacacagaaagagtttgtagaaacgcaaaaaggccatccgtcaggggccttctgcttagtttgatgcctggcagttccctactctcgccttccgcttcctcgctcactgactcgctgcgctcggtcgttcggctgcggcgagcggtatcagctcactcaaaggcggtaatacggttatccacagaatcaggggataacgcaggaaagaacatgtgagcaaaaggccagcaaaaggccaggaaccgtaaaaaggccgcgttgctggcgtttttccataggctccgcccccctgacgagcatcacaaaaatcgacgctcaagtcagaggtggcgaaacccgacaggactataaagataccaggcgtttccccctggaagctccctcgtgcgctctcctgttccgaccctgccgcttaccggatacctgtccgcctttctcccttcgggaagcgtggcgctttctcatagctcacgctgtaggtatctcagttcggtgtaggtcgttcgctccaagctgggctgtgtgcacgaaccccccgttcagcccgaccgctgcgccttatccggtaactatcgtcttgagtccaacccggtaagacacgacttatcgccactggcagcagccactggtaacaggattagcagagcgaggtatgtaggcggtgctacagagttcttgaagtggtgggctaactacggctacactagaagaacagtatttggtatctgcgctctgctgaagccagttaccttcggaaaaagagttggtagctcttgatccggcaaacaaaccaccgctggtagcggtggtttttttgtttgcaagcagcagattacgcgcagaaaaaaaggatctcaagaagatcctttgatcttttctacggggtctgacgctcagtggaacgacgcgcgcgtaactcacgttaagggattttggtcatgagcttgcgccgtcccgtcaagtcagcgtaatgctctgcttttagaaaaactcatcgagcatcaaatgaaactgcaatttattcatatcaggattatcaataccatatttttgaaaaagccgtttctgtaatgaaggagaaaactcaccgaggcagttccataggatggcaagatcctggtatcggtctgcgattccgactcgtccaacatcaatacaacctattaatttcccctcgtcaaaaataaggttatcaagtgagaaatcaccatgagtgacgactgaatccggtgagaatggcaaaagtttatgcatttctttccagacttgttcaacaggccagccattacgctcgtcatcaaaatcactcgcatcaaccaaaccgttattcattcgtgattgcgcctgagcgaggcgaaatacgcgatcgctgttaaaaggacaattacaaacaggaatcgagtgcaaccggcgcaggaacactgccagcgcatcaacaatattttcacctgaatcaggatattcttctaatacctggaacgctgtttttccggggatcgcagtggtgagtaaccatgcatcatcaggagtacggataaaatgcttgatggtcggaagtggcataaattccgtcagccagtttagtctgaccatctcatctgtaacatcattggcaacgctacctttgccatgtttcagaaacaactctggcgcatcgggcttcccatacaagcgatagattgtcgcacctgattgcccgacattatcgcgagcccatttatacccatataaatcagcatccatgttggaatttaatcgcggcctcgacgtttcccgttgaatatggctcatattcttcctttttcaatattattgaagcatttatcagggttattgtctcatgagcggatacatatttgaatgtatttagaaaaataaacaaataggggtcagtgttacaaccaattaaccaattctgaacattatcgcgagcccatttatacctgaatatggctcataacaccccttgtttgcctggcggcagtagcgcggtggtcccacctgaccccatgccgaactcagaagtgaaacgccgtagcgccgatggtagtgtggggactccccatgcgagagtagggaactgccaggcatcaaataaaacgaaaggctcagtcgaaagactgggcctttcgcccgggctaattagggggtgtcgcccttattcgactctatagtgaagttcctattctctagaaagtataggaacttctgaagt

SEQ ID NO: 84 - DNA, 15025 bp, Artificial sequence
  synthetic Dox-rapamycin inducible GAG POL ENV
gatatctataacaagaaaatatatatataataagttatcacgtaagtagaacatgaaataacaatataattatcgtatgagttaaatcttaaaagtcacgtaaaagataatcatgcgtcattttgactcacgcggtcgttatagttcaaaatcagtgacacttaccgcattgacaagcacgcctcacgggagctccaagcggcgactgagatgtcctaaatgcacagcgacggattcgcgctatttagaaagagagagcaatatttcaagaatgcatgcgtcaattttacgcagactatctttctagggttaagacggatcgggagatctcccgatcccctatggtgcactctcagtacaatctgctctgatgccgcatagttaagccagtatctgctccctgcttgtgtgttggaggtcgctgagtagtgcgcgagcaaaatttaagctacaacaaggcaaggcttgaccgacaattgcatgaagaatctgcttagggttaggcgttttgaagttcctatactttctagagaataggaacttcggaataggaacttcggatgcaatttcctcattttattaggaaaggacagtgggagtggcaccttccagggtcaaggaaggcacgggggaggggcaaacaacagatggctggcaactagaaggcacagcgttagtgatacttgtgggccagggcattagccacaccagccaccactttctgataggcagcctgcactggtggggtgaattccgcggaagcttgtgtaattgttaatttctctgtcccactccatccaggtcgtgtgattccaaatctgttccagagatttattactccaactagcattccaaggcacagcagtggtgcaaatgagttttccagagcaaccccaaatccccaggagctgttgatcctttaggtatctttccacagccaggattcttgcctggagctgcttgatgccccagactgtgagttgcaacagatgctgttgcgcctcaatagccctcagcaaattgttctgctgctgcactataccagacaataattgtctggcctgtaccgtcagcgtcattgacgctgcgcccatagtgcttcctgctgctcccaagaacccaaggaacaaagctcctgcggccgctccggaattccatgtgttaatcctcatcctgtctacttgccacacaatcatcacctgccatctgttttccataatccctgatgatctttgcttttcttcttggcactacttttatgtcactattatcttgtattactactgccccttcacctttccagaggagctttgctggtcctttccaaactggatctctgctgtccctgtaataaacccgaaaattttgaatttttgtaatttgtttttgtaattctttagtttgtatgtctgttgctattatgtctactattctttcccctgcactgtaccccccaatccccccttttcttttaaaattgtggatgaatactgccatttgtactgctgtcttaagatgttcagcctgatctcttacctgtcctataattttctttaattctttattcatagattctattactccttgactttggggattgtagggaatgccaaattcctgcttgatccccgcccaccaacaggcggccttaactgtagtactggtgaaattgctgccattgtctgtatgtactgtttttactggccatcttcctgctaattttaagaggaagtatgctgtttcttgccctgtctctgctggaattacttctgcttctatatatccactggctacatgaactgctaccaagataacttttccttctaaatgtgtacaatctagctgccatattcctgggctacagtctacttgtccatgcatggcttccccttttagctgacatttatcacagctggctactatttcttttgctactacaggtggtaggttaaaatcactagccattgctctccaattactgtgatatttctcatgttcttcttgggccttatctattccatctaaaaatagtactttcctgattccagcactgaccaatttatctacttgttcatttcctccaattcctttgtgtgctggtacccatgccaggtagactttttccttttttattaactgctctattatttgactgactaactctgattcactcttatctggttgtgcttgaatgattcccaatgcatattgtgagtctgtcactatgtttacttctaatcccgaatcctgcaaagctagatgaattgcttgtaactcagtcttctgatttgttgtgtccgttagggggacaactttttgtcttcctctgtcagttacatatcctgcttttcctaatttagtttccctattggctgccccatctacatagaaagtttctgctcctattatgggttctttctctaactggtaccataacttcactaagggaggggtattgacaaactcccactcaggaatccaggtggcttgccaatactctgtccaccatgcttcccatgtttccttttgtatgggtaatttaaatttaggagtctttccccatattactatgctttctgtggctattttttgtactgcctctgttaattgtttcacatcattagtgtgggcacccttcattcttgcatactttcctgttttcagatttttaaatggctcttgataaatttgatatgtccattggccttgcccctgcttctgtatttctgctattaagtcttttgatgggtcataatacactccatgtaccggttcttttagaatctccctgttttctgccagttctagctctgcttcttctgttagtggtactacttctgttagtgctttggttcccctaagaagtttacataattgccttactttaatccctgcataaatctgacttgcccaattcaattttcccactaatttctgtatgtcattgacagtccagctgtccttttctggcagcactataggctgtactgtccatttatcaggatggagttcataacccatccaaaggaatggaggttctttctgatgttttttgtctggtgtggtaaatccccacctcaacagatgttgtctcagttcctctatttttgttctatgctgccctatttctaagtcagatcctacatacaaatcatccatgtattgatagatgactatgtctggattttgttttctaaaaggctctaagatttttgtcatgctacactggaatattgctggtgatcctttccatccctgtggaagcacattgtactgatatctaatccctggtgtctcattgtttatactaggtatggtaaatgcagtatacttcctgaagtctttatctaagggaactgaaaaatatgcatcgcccacatccagtactgttactgattttttctgttttaaccctgcaggatgtggtattcctaattgaacttcccagaaatcttgagttctcttattaagttctctgaaatctactaattttctccatttagtactgtcttttttctttatggcaaatactggagtattgtatggattttcaggcccaatttttgaaatttttccttccttttccatttctgtacaaatttctactaatgcttttattttttcttctgtcaatggccattgtttaacttttgggccatccattcctggctttaattttactggtacagtctcaataggactaatgggaaaatttaaagtgcagccaatctgagtcaacagatttcttccaattatgttgacaggtgtaggtcctactaatactgtacctatagctttatgtccgcagatttctatgagtatctgatcatactgtcttactttgataaaacctccaattccccctatcatttttggtttccatcttcctggcaaattcatttcttctaatactgtatcatctgctcctgtatctaatagagcttcctttaattgcccccctatctttattgtgacgaggggtcgctgccaaagagtgatctgagggaagctaaaggatacagttccttgtctatcggctcctgcttctgagagggagttgttgtctcttccccaaacctgaagctctcttctggtggggctgttggctctggtctgctctgaagaaaattccctggccttcccttgtgggaaggccagatcttccctaaaaaattagcctgtctctcagtacaatctttcatttggtgtccttcctttccacatttccaacagccctttttcctaggggccctgcaatttttggctatgtgcccttctttgccacaattgaaacacttaacagtctttctttggttcctaaaattgcctttctgtatcattatggtagctggatttgttacttggctcattgcttcagccaaaactcttgctttatggccgggtccccccactccctgacatgctgtcatcatttcttctagtgtcgctcctggtcccaatgcttttaaaatagtcttacaatctgggttcgcattttggaccaacaaggtttctgtcatccaattttttacctcttgtgaagcttgctcggctcttagagttttatagaatcggtctacatagtctctaaagggttcctttggtccttgtcttatgtccagaatgctggtagggctatacattcttactattttatttaatcccaggattatccatcttttatagatttctcctactgggataggtggattatgtgtcatccatcctatttgttcctgaagggtactagtagttcctgctatgtcacttccccttggttctctcatctggcctggtgcaataggccctgcatgcactggatgcactctatcccattctgcagcttcctcattgatggtctcttttaacatttgcatggctgcttgatgtccccccactgtgtttagcatggtgtttaaatcttgtggggtggctccttctgataatgctgaaaacatgggtatcacttctgggctgaaagccttctcttctactacttttacccatgcatttaaagttctaggtgatatggcctgatgtaccatttgcccctggatgttctgcactatagggtaattttggctgacctgattgctgtgtcctgtgtcagctgctgcttgctgtgcttttttcttacttttgttttgctcttcctctatcttgtctaaagcttccttggtgtcttttatctctatcctttgatgcacacaatagagggttgctactgtattatataatgatctaagttcttctgatcctgtctgaagggatggttgtagctgtcccagtatttgtctacagccttctgatgtttctaacaggccaggattaactgcgaatcgttctagctccctgcttgcccatactatatgttttaatttatattttttctttccccctggccttaaccgaattttttcccatcgatctaattctcccccgcttaatactgacgctctcgcacccatggcggcggcagatctcgaattcagatctcacgtgctttgccaaagtgatgggccagcacacagaccagcacgttgcccaggagctgtgggaggaagataagaggtatgaacatgattagcaaaagggcctagcttggactcagaataatccagccttatcccaaccataaaataaaagcagaatggtagctggattgtagctgctattagcaatatgaaacctcttacatcagttacaatttatatgcagaaatatttatatgcagaaatattgctattgccttaacccagaaattatcactgttattctttagaatggtgcaaagaggcatgatacattgtatcattattgccctgaaagaaagagattagggaaagtattagaaataagataaacaaaaaagtatattaaaagaagaaagcattttttaaaattacaaatgcaaaattaccctgatttggtcaatatgtgtaccctgttacttctccccttcctatgacatgaacttaaccatagaaaagaaggggaaagaaaacatcaagggtcccatagactcaccctgaagttctcaggatccgagctcggtaccacatgtaagcttcgaggggaggctggatcggtcccggtgtcttctatggaggtcaaaacagcgtggatggcgtctccaggcgatctgacggttcactaaacgctgcttcgcgatgtacgggccagatatacgcgttgcgatctgacggttcactaaacgagctctgcttatataggcctcccaccgtacacgccacctcgacatactcgagtttactccctatcagtgatagagaacgtatgaagagtttactccctatcagtgatagagaacgtatgcagactttactccctatcagtgatagagaacgtataaggagtttactccctatcagtgatagagaacgtatgaccagtttactccctatcagtgatagagaacgtatctacagtttactccctatcagtgatagagaacgtatatccagtttactccctatcagtgatagagaacgtataagctttaggcgtgtacggtgggcgcctataaaagcagagctcgtttagtgaaccgtcagatcgcctggagcaattccacaacacttttgtcttataccaactttccgtaccacttcctaccctcgtaaatcgtcgacgagctcgtttagtgaaccgtcagatcgcctggagacgccctcgaagccgcggtgcgggtgccagggcgtgcccttgggctccatgtccatcatgggtctcaaggtgaacgtctctgccatattcatggcagtactgttaactctccaaacacccaccggtcaaatccattggggcaatctctctaagataggggtggtaggaataggaagtgcaagctacaaagttatgactcgttccagccatcaatcattagtcataaaattaatgcccaatataactctcctcaataactgcacgagggtagagattgcagaatacaggagactactgagaacagttttggaaccaattagagatgcacttaatgcaatgacccagaatataagaccggttcagagtgtagcttcaagtaggagacacaagagatttgcgggagtagtcctggcaggtgcggccctaggcgttgccacagctgctcagataacagccggcattgcacttcaccagtccatgctgaactctcaagccatcgacaatctgagagcgagcctggaaactactaatcaggcaattgaggcaatcagacaagcagggcaggagatgatattggctgttcagggtgtccaagactacatcaataatgagctgataccgtctatgaaccaactatcttgtgatttaatcggccagaagctcgggctcaaattgctcagatactatacagaaatcctgtcattatttggccccagcttacgggaccccatatctgcggagatatctatccaggctttgagctatgcgcttggaggagacatcaataaggtgttagaaaagctcggatacagtggaggtgatttactgggcatcttagagagcagaggaataaaggcccggataactcacgtcgacacagagtcctacttcattgtcctcagtatagcctatccgacgctgtccgagattaagggggtgattgtccaccggctagagggggtctcgtacaacataggctctcaagagtggtataccactgtgcccaagtatgttgcaacccaagggtaccttatctcgaattttgatgagtcatcgtgtactttcatgccagaggggactgtgtgcagccaaaatgccttgtacccgatgagtcctctgctccaagaatgcctccgggggtccaccaagtcctgtgctcgtacactcgtatccgggtcttttgggaaccggttcattttatcacaagggaacctaatagccaattgtgcatcaatcctttgcaagtgttacacaacaggaacgatcattaatcaagaccctgacaagatcctaacatacattgctgccgatcactgcccggtagtcgaggtgaacggcgtgaccatccaagtcgggagcaggaggtatccagacgctgtgtacttgcacagaattgacctcggtcctcccatatcattggagaggttggacgtagggacaaatctggggaatgcaattgctaagttggaggatgccaaggaattgttggagtcatcggaccagatattgaggagtatgaaaggtttatcgagcactagcatagtctacatcctgattgcagtgtgtcttggagggttgatagggatccccgctttaatatgttgctgcagggggcgttgacccctctccctcccccccccctaacgttactggccgaagccgcttggaataaggccggtgtgcgtttgtctatatgttattttccaccatattgccgtcttttggcaatgtgagggcccggaaacctggccctgtcttcttgacgagcattcctaggggtctttcccctctcgccaaaggaatgcaaggtctgttgaatgtcgtgaaggaagcagttcctctggaagcttcttgaagacaaacaacgtctgtagcgaccctttgcaggcagcggaaccccccacctggcgacaggtgcctctgcggccaaaagccacgtgtataagatacacctgcaaaggcggcacaaccccagtgccacgttgtgagttggatagttgtggaaagagtcaaatggctctcctcaagcgtattcaacaaggggctgaaggatgcccagaaggtaccccattgtatgggatctgatctggggcctcggtacacatgctttacatgtgtttagtcgaggttaaaaaaacgtctaggccccccgaaccacggggacgtggttttcctttgaaaaacacgatgataatatggccacaaccatgggaagtaggatagtcattaacagagaacatcttatgattgatagaccttatgttttgctggctgttctgtttgtcatgtttctgagcttgatcgggttgctagccattgcaggcattagacttcatcgggcagccatctacaccgcagagatccataaaagcctcagcaccaatctagatgtaactaactcaatcgagcatcaggtcaaggacgtgctgacaccactcttcaaaatcatcggtgatgaagtgggcctgaggacacctcagagattcactgacctagtgaaattcatctctgacaagattaaattccttaatccggatagggagtacgacttcagagatctcacttggtgtatcaacccgccagagagaatcaaattggattatgatcaatactgtgcagatgtggctgctgaagagctcatgaatgcattggtgaactcaactctactggagaccagaacaaccaatcagttcctagctgtctcaaagggaaactgctcagggcccactacaatcagaggtcaattctcaaacatgtcgctgtccctgttagacttgtatttaggtcgaggttacaatgtgtcatctatagtcactatgacatcccagggaatgtatgggggaacttacctagtggaaaagcctaatctgagcagcaaaaggtcagagttgtcacaactgagcatgtaccgagtgtttgaagtaggtgttatcagaaatccgggtttgggggctccggtgttccatatgacaaactatcttgagcaaccagtcagtaatgatctcagcaactgtatggtggctttgggggagctcaaactcgcagccctttgtcacggggaagattctatcacaattccctatcagggatcagggaaaggtgtcagcttccagctcgtcaagctaggtgtctggaaatccccaaccgacatgcaatcctgggtccccttatcaacggatgatccagtgatagacaggctttacctctcatctcacagaggtgttatcgctgacaaycaagcaaaatgggctgtcccgacaacacgaacagatgacaagttgcgaatggagacatgcttccaacaggcgtgtaagggtaaaatccaagcactctgcgagaatcccgagtgggcaccattgaaggataacaggattccttcatacggggtcttgtctgttgatctgagtctgacagttgagcttaaaatcaaaattgcttcgggattcgggccattgatcacacacggttcagggatggacctatacaaatccaaccacaacaatgtgtattggctgactatcccrccaatgaagaacctagccttaggtgtaatcaacacattggagtggataccgagattcaaggttagtccctacctcttcamtgtcccaattaaggaagcaggcgaagactgccatgccccaacatacctacctgcggaggtggatggtgatgtcaaactcagttccaatctggtgattctacctggtcaagatctccaatatgttttggcaacctacgatacttccagggttgaacatgctgtggtttattacgtttacagcccaagccgctcattttcttacttttatccttttaggttgcctataaagggggtccccatcgaattacaagtggaatgcttcacatgggaccaaaaactctggtgccgtcacttctgtgtgcttgcggactcagaatctggtggacatatcactcactctgggatggtgggcatgggagtcagctgcacagtcacccgggaagatggaaccaatcgcagatagggctgctagtgaacyaatcwcatgatgtcacccagacatcaggcatacccactagtgtgaaatagacatcagaattaagaaaaatgggctccccgggcgcgtactccacctcacccatcatccacgctcggcaataaaaagacagaataaaacgcacgggtgttgggtcgtttgttcgccgggcgcgtactccacctcacccatcatccacgctgttttatggatagcactgagaacgtcatcaagcccttcatgcgcttcaaggtgcacatggagggctccgtgaacggccacgagttcgagatcgagggcgagggcgagggcaagccctacgagggcacccagaccgccaagctgcaggtgaccaagggcggccccctgcccttcgcctgggacatcctgtccccccagttccagtacggctccaaggtgtacgtgaagcaccccgccgacatccccgactacaagaagctgtccttccccgagggcttcaagtgggagcgcgtgatgaacttcgaggacggcggcgtggtgaccgtgacccaggactcctccctgcaggacggcaccttcatctaccacgtgaagttcatcggcgtgaacttcccctccgacggccccgtaatgcagaagaagactctgggctgggagccctccaccgagcgcctgtacccccgcgacggcgtgctgaagggcgagatccacaaggcgctgaagctgaagggcggcggccactacctggtggagttcaagtcaatctacatggccaagaagcccgtgaagctgcccggctactactacgtggactccaagctggacatcacctcccacaacgaggactacaccgtggtggagcagtacgagcgcgccgaggcccgccaccacctgttccagtaggacctccatagaagacaccgggaccgatccaataacttcgtatagcatacattatacgaagttatgcctccggactctagcgtttaaacttaagcttggtaccgagctcggatccactagtccagtgtggtggaattctgcagatatccagcacagtggcggccgctcgagtctagagggcccgtttaaacccgctgatcagcctcgactgtgccttctagttgccagccatctgttgtttgcccctcccccgtgccttccttgaccctggaaggtgccactcccactgtcctttcctaataaaatgaggaaattgcatcgcattgtctgagtaggtgtcattctattctggggggtggggtggggcaggacagcaagggggaggattgggaagacaatagcaggcatgctggggatgcggtgggctctatggcttctgaggcggaaagttaaccctagaaagataatcatattgtgacgtacgttaaagataatcatgcgtaaaattgacgcatgtgttttatcggtctgtatatcgaggtttatttattaatttgaatagatattaagttttattatatttacacttacatactaataataaattcaacaaacaatttatttatgtttatttatttattaaaaaaaaacaaaaactcaaaatttcttctataaagtaacaaaaaccagctggggctcgaagttcctatactttctagagaataggaacttctatagtgagtcgaataagggcgacacaaaatttattctaaatgcataataaatactgataacatcttatagtttgtattatattttgtattatcgttgacatgtataattttgatatcaaaaactgattttccctttattattttcgagatttattttcttaattctctttaacaaactagaaatattgtatatacaaaaaatcataaataatagatgaatagtttaattataggtgttcatcaatcgaaaaagcaacgtatcttatttaaagtgcgttgcttttttctcatttataaggttaaataattctcatatatcaagcaaagtgacaggcgcccttaaatattctgacaaatgctctttccctaaactccccccataaaaaaacccgccgaagcgggtttttacgttatttgcggattaacgattactcgttatcagaaccgcccagggggcccgagcttaagactggccgtcgttttacaacacagaaagagtttgtagaaacgcaaaaaggccatccgtcaggggccttctgcttagtttgatgcctggcagttccctactctcgccttccgcttcctcgctcactgactcgctgcgctcggtcgttcggctgcggcgagcggtatcagctcactcaaaggcggtaatacggttatccacagaatcaggggataacgcaggaaagaacatgtgagcaaaaggccagcaaaaggccaggaaccgtaaaaaggccgcgttgctggcgtttttccataggctccgcccccctgacgagcatcacaaaaatcgacgctcaagtcagaggtggcgaaacccgacaggactataaagataccaggcgtttccccctggaagctccctcgtgcgctctcctgttccgaccctgccgcttaccggatacctgtccgcctttctcccttcgggaagcgtggcgctttctcatagctcacgctgtaggtatctcagttcggtgtaggtcgttcgctccaagctgggctgtgtgcacgaaccccccgttcagcccgaccgctgcgccttatccggtaactatcgtcttgagtccaacccggtaagacacgacttatcgccactggcagcagccactggtaacaggattagcagagcgaggtatgtaggcggtgctacagagttcttgaagtggtgggctaactacggctacactagaagaacagtatttggtatctgcgctctgctgaagccagttaccttcggaaaaagagttggtagctcttgatccggcaaacaaaccaccgctggtagcggtggtttttttgtttgcaagcagcagattacgcgcagaaaaaaaggatctcaagaagatcctttgatcttttctacggggtctgacgctcagtggaacgacgcgcgcgtaactcacgttaagggattttggtcatgagcttgcgccgtcccgtcaagtcagcgtaatgctctgcttttagaaaaactcatcgagcatcaaatgaaactgcaatttattcatatcaggattatcaataccatatttttgaaaaagccgtttctgtaatgaaggagaaaactcaccgaggcagttccataggatggcaagatcctggtatcggtctgcgattccgactcgtccaacatcaatacaacctattaatttcccctcgtcaaaaataaggttatcaagtgagaaatcaccatgagtgacgactgaatccggtgagaatggcaaaagtttatgcatttctttccagacttgttcaacaggccagccattacgctcgtcatcaaaatcactcgcatcaaccaaaccgttattcattcgtgattgcgcctgagcgaggcgaaatacgcgatcgctgttaaaaggacaattacaaacaggaatcgagtgcaaccggcgcaggaacactgccagcgcatcaacaatattttcacctgaatcaggatattcttctaatacctggaacgctgtttttccggggatcgcagtggtgagtaaccatgcatcatcaggagtacggataaaatgcttgatggtcggaagtggcataaattccgtcagccagtttagtctgaccatctcatctgtaacatcattggcaacgctacctttgccatgtttcagaaacaactctggcgcatcgggcttcccatacaagcgatagattgtcgcacctgattgcccgacattatcgcgagcccatttatacccatataaatcagcatccatgttggaatttaatcgcggcctcgacgtttcccgttgaatatggctcatattcttcctttttcaatattattgaagcatttatcagggttattgtctcatgagcggatacatatttgaatgtatttagaaaaataaacaaataggggtcagtgttacaaccaattaaccaattctgaacattatcgcgagcccatttatacctgaatatggctcataacaccccttgtttgcctggcggcagtagcgcggtggtcccacctgaccccatgccgaactcagaagtgaaacgccgtagcgccgatggtagtgtggggactccccatgcgagagtagggaactgccaggcatcaaataaaacgaaaggctcagtcgaaagactgggcctttcgcccgggctaattagggggtgtcgcccttattcgactctatagtgaagttcctattctctagaaagtataggaacttctgaagt

SEQ ID NO: 85 - DNA, 6584 bp, Artificial sequence
  synthetic Rapamycin-inducible TET activator
gatatctataacaagaaaatatatatataataagttatcacgtaagtagaacatgaaataacaatataattatcgtatgagttaaatcttaaaagtcacgtaaaagataatcatgcgtcattttgactcacgcggtcgttatagttcaaaatcagtgacacttaccgcattgacaagcacgcctcacgggagctccaagcggcgactgagatgtcctaaatgcacagcgacggattcgcgctatttagaaagagagagcaatatttcaagaatgcatgcgtcaattttacgcagactatctttctagggttaagacggatcgggagatctcccgatcccctatggtgcactctcagtacaatctgctctgatgccgcatagttaagccagtatctgctccctgcttgtgtgttggaggtcgctgagtagtgcgcgagcaaaatttaagctacaacaaggcaaggcttgaccgacaattgcatgaagaatctgcttagggttaggcgttttgcgctgcttcgcgatgtacgggccagatatacgcgttctccatagaagacaccgaataaaatatctttattttcattacatctgtgtgttggttttttgtgtgaatcgatagtactaacatacgctctccatcaaaacaaaacgaaacaaaacaaactagcaaaataggctgtccccagtgcaagtgcaggtgccagaacatttctctggaccgatccaataacttcgtatagcatacattatacgaagttatgcctccggactctagcgttttagttattactagcgctaccggactcagatctcgagctcaagcttcgaattctgcagtcgacggtaccgcggcttacgcgtgctagctaatgatgggcgctcgagtaatgatgggcggtcgactaatgatgggcgctcgagtaatgatgggcgtctagctaatgatgggcgctcgagtaatgatgggcggtcgactaatgatgggcgctcgagtaatgatgggcgtctagctaatgatgggcgctcgagtaatgatgggcggtcgactaatgatgggcgctcgagtaatgatgggcgtctagaacgcgaattaattcaacattttgacacccccataatatttttccagaattaacagtataaattgcatctcttgttcaagagttccctatcactctctttaatcactactcacagtaacctcaactcctgccacaagcttgccctgcagcgggaattccaaacttaagcttggtaccgagctcggatccactagtccagtgtggtggaattctgcagatatccagcacagtggcggccgctcgagtctagagggcccgtttaaacccgctgatcaatgtctagactggacaagagcaaagtcataaactctgctctggaattactcaatggagtcggtatcgaaggcctgacgacaaggaaactcgctcaaaagctgggagttgagcagcctaccctgtactggcacgtgaagaacaagcgggccctgctcgatgccctgccaatcgagatgctggacaggcatcatacccactcctgccccctggaaggcgagtcatggcaagactttctgcggaacaacgccaagtcataccgctgtgctctcctctcacatcgcgacggggctaaagtgcatctcggcacccgcccaacagagaaacagtacgaaaccctggaaaatcagctcgcgttcctgtgtcagcaaggcttctccctggagaacgcactgtacgctctgtccgccgtgggccactttacactgggctgcgtattggaggaacaggagcatcaagtagcaaaagaggaaagagagacacctaccaccgattctatgcccccacttctgaaacaagcaattgagctgttcgaccggcagggagccgaacctgccttccttttcggcctggaactaatcatatgtggcctggagaaacagctaaagtgcgaaagcggcgggccgaccgacgcccttgacgattttgacttagacatgctcccagccgatgcccttgacgactttgaccttgatatgctgcctgctgacgctcttgacgattttgaccttgacatgctccccgggtaagtccctcccccccccctaacgttactggccgaagccgcttggaataaggccggtgtgcgtttgtctatatgttattttccaccatattgccgtcttttggcaatgtgagggcccggaaacctggccctgtcttcttgacgagcattcctaggggtctttcccctctcgccaaaggaatgcaaggtctgttgaatgtcgtgaaggaagcagttcctctggaagcttcttgaagacaaacaacgtctgtagcgaccctttgcaggcagcggaaccccccacctggcgacaggtgcctctgcggccaaaagccacgtgtataagatacacctgcaaaggcggcacaaccccagtgccacgttgtgagttggatagttgtggaaagagtcaaatggctctcctcaagcgtattcaacaaggggctgaaggatgcccagaaggtaccccattgtatgggatctgatctggggcctcggtgcacatgctttacatgtgtttagtcgaggttaaaaaacgtctaggccccccgaaccacggggacgtggttttcctttgaaaaacacgatgataaatggatagcactgagaacgtcatcaagcccttcatgcgcttcaaggtgcacatggagggctccgtgaacggccacgagttcgagatcgagggcgagggcgagggcaagccctacgagggcacccagaccgccaagctgcaggtgaccaagggcggccccctgcccttcgcctgggacatcctgtccccccagttccagtacggctccaaggtgtacgtgaagcaccccgccgacatccccgactacaagaagctgtccttccccgagggcttcaagtgggagcgcgtgatgaacttcgaggacggcggcgtggtgaccgtgacccaggactcctccctgcaggacggcaccttcatctaccacgtgaagttcatcggcgtgaacttcccctccgacggccccgtaatgcagaagaagactctgggctgggagccctccaccgagcgcctgtacccccgcgacggcgtgctgaagggcgagatccacaaggcgctgaagctgaagggcggcggccactacctggtggagttcaagtcaatctacatggccaagaagcccgtgaagctgcccggctactactacgtggactccaagctggacatcacctcccacaacgaggactacaccgtggtggagcagtacgagcgcgccgaggcccgccaccacctgttccagtagctcgactgtgccttctagttgccagccatctgttgtttgcccctcccccgtgccttccttgaccctggaaggtgccactcccactgtcctttcctaataaaatgaggaaattgcatcgcattgtctgagtaggtgtcattctattctggggggtggggtggggcaggacagcaagggggaggattgggaagacaatagcaggcatgctggggatgcggtgggctctatggcttctgaggcggaaagttaaccctagaaagataatcatattgtgacgtacgttaaagataatcatgcgtaaaattgacgcatgtgttttatcggtctgtatatcgaggtttatttattaatttgaatagatattaagttttattatatttacacttacatactaataataaattcaacaaacaatttatttatgtttatttatttattaaaaaaaaacaaaaactcaaaatttcttctataaagtaacaaaaaccagctggggctcgaagttcctatactttctagagaataggaacttctatagtgagtcgaataagggcgacacaaaatttattctaaatgcataataaatactgataacatcttatagtttgtattatattttgtattatcgttgacatgtataattttgatatcaaaaactgattttccctttattattttcgagatttattttcttaattctctttaacaaactagaaatattgtatatacaaaaaatcataaataatagatgaatagtttaattataggtgttcatcaatcgaaaaagcaacgtatcttatttaaagtgcgttgcttttttctcatttataaggttaaataattctcatatatcaagcaaagtgacaggcgcccttaaatattctgacaaatgctctttccctaaactccccccataaaaaaacccgccgaagcgggtttttacgttatttgcggattaacgattactcgttatcagaaccgcccagggggcccgagcttaagactggccgtcgttttacaacacagaaagagtttgtagaaacgcaaaaaggccatccgtcaggggccttctgcttagtttgatgcctggcagttccctactctcgccttccgcttcctcgctcactgactcgctgcgctcggtcgttcggctgcggcgagcggtatcagctcactcaaaggcggtaatacggttatccacagaatcaggggataacgcaggaaagaacatgtgagcaaaaggccagcaaaaggccaggaaccgtaaaaaggccgcgttgctggcgtttttccataggctccgcccccctgacgagcatcacaaaaatcgacgctcaagtcagaggtggcgaaacccgacaggactataaagataccaggcgtttccccctggaagctccctcgtgcgctctcctgttccgaccctgccgcttaccggatacctgtccgcctttctcccttcgggaagcgtggcgctttctcatagctcacgctgtaggtatctcagttcggtgtaggtcgttcgctccaagctgggctgtgtgcacgaaccccccgttcagcccgaccgctgcgccttatccggtaactatcgtcttgagtccaacccggtaagacacgacttatcgccactggcagcagccactggtaacaggattagcagagcgaggtatgtaggcggtgctacagagttcttgaagtggtgggctaactacggctacactagaagaacagtatttggtatctgcgctctgctgaagccagttaccttcggaaaaagagttggtagctcttgatccggcaaacaaaccaccgctggtagcggtggtttttttgtttgcaagcagcagattacgcgcagaaaaaaaggatctcaagaagatcctttgatcttttctacggggtctgacgctcagtggaacgacgcgcgcgtaactcacgttaagggattttggtcatgagcttgcgccgtcccgtcaagtcagcgtaatgctctgcttttagaaaaactcatcgagcatcaaatgaaactgcaatttattcatatcaggattatcaataccatatttttgaaaaagccgtttctgtaatgaaggagaaaactcaccgaggcagttccataggatggcaagatcctggtatcggtctgcgattccgactcgtccaacatcaatacaacctattaatttcccctcgtcaaaaataaggttatcaagtgagaaatcaccatgagtgacgactgaatccggtgagaatggcaaaagtttatgcatttctttccagacttgttcaacaggccagccattacgctcgtcatcaaaatcactcgcatcaaccaaaccgttattcattcgtgattgcgcctgagcgaggcgaaatacgcgatcgctgttaaaaggacaattacaaacaggaatcgagtgcaaccggcgcaggaacactgccagcgcatcaacaatattttcacctgaatcaggatattcttctaatacctggaacgctgtttttccggggatcgcagtggtgagtaaccatgcatcatcaggagtacggataaaatgcttgatggtcggaagtggcataaattccgtcagccagtttagtctgaccatctcatctgtaacatcattggcaacgctacctttgccatgtttcagaaacaactctggcgcatcgggcttcccatacaagcgatagattgtcgcacctgattgcccgacattatcgcgagcccatttatacccatataaatcagcatccatgttggaatttaatcgcggcctcgacgtttcccgttgaatatggctcatattcttcctttttcaatattattgaagcatttatcagggttattgtctcatgagcggatacatatttgaatgtatttagaaaaataaacaaataggggtcagtgttacaaccaattaaccaattctgaacattatcgcgagcccatttatacctgaatatggctcataacaccccttgtttgcctggcggcagtagcgcggtggtcccacctgaccccatgccgaactcagaagtgaaacgccgtagcgccgatggtagtgtggggactccccatgcgagagtagggaactgccaggcatcaaataaaacgaaaggctcagtcgaaagactgggcctttcgcccgggctaattagggggtgtcgcccttattcgactctatagtgaagttcctattctctagaaagtataggaacttctgaagt

SEQ ID NO: 86 - DNA, 11528 bp, Artificial sequence
  synthetic Rapamycin inducer inducible REV srcVpx
gatatctataacaagaaaatatatatataataagttatcacgtaagtagaacatgaaataacaatataattatcgtatgagttaaatcttaaaagtcacgtaaaagataatcatgcgtcattttgactcacgcggtcgttatagttcaaaatcagtgacacttaccgcattgacaagcacgcctcacgggagctccaagcggcgactgagatgtcctaaatgcacagcgacggattcgcgctatttagaaagagagagcaatatttcaagaatgcatgcgtcaattttacgcagactatctttctagggttaagacggatcgggagatctcccgatcccctatggtgcactctcagtacaatctgctctgatgccgcatagttaagccagtatctgctccctgcttgtgtgttggaggtcgctgagtagtgcgcgagcaaaatttaagctacaacaaggcaaggcttgaccgacaattgcatgaagaatctgcttagggttaggcgttttgcgctgcttcgcgatgtacgggccagatatacgcgttgacattgattattgactagttattaatagtaatcaattacggggtcattagttcatagcccatatatggagttccgcgttacataacttacggtaaatggcccgcctggctgaccgcccaacgacccccgcccattgacgtcaataatgacgtatgttcccatagtaacgccaatagggactttccattgacgtcaatgggtggagtatttacggtaaactgcccacttggcagtacatcaagtgtatcatatgccaagtacgccccctattgacgtcaatgacggtaaatggcccgcctggcattatgcccagtacatgaccttatgggactttcctacttggcagtacatctacgtattagtcatcgctattaccatggtgatgcggttttggcagtacatcaatgggcgtggatagcggtttgactcacggggatttccaagtctccaccccattgacgtcaatgggagtttgttttggaaccaaaatcaacgggactttccaaaatgtcgtaacaactccgccccattgacgcaaatgggcggtaggcgtgtacggtgggaggtctatataagcagagctcggcattgattattgactagttattaatagtaatcaattacggggtcattagttcatagcccatatatggagttccgcgttacataacttacggtaaatggcccgcctggctgaccgcccaacgacccccgcccattgacgtcaataatgacgtatgttcccatagtaacgccaatagggactttccattgacgtcaatgggtggagtatttacggtaaactgcccacttggcagtacatcaagtgtatcatatgccaagtccgccccctattgacgtcaatgacggtaaatggcccgcctggcattatgcccagtacatgaccttacgggactttcctacttggcagtacatctacgtattagtcatcgctattaccatggtgatgcggttttggcagtacaccaatgggcgtggatagcggtttgactcacggggatttccaagtctccaccccattgacgtcaatgggagtttgttttggcaccaaaatcaacgggactttccaaaatgtcgtaacaactgcgatcgcccgccccgttgacgcaaatgggcggtaggcgtgtacggtgggaggtctatataagcagagctcgtttagtgaaccgtcagatcactagaagctttattgcggtagtttatcacagttaaattgctaacgcagtcagtgcttctgacacaacagtctcgaacttaagctgcagtgactctcttaaggtagccttgcagaagttggtcgtgaggcactgggcaggtaagtatcaaggttacaagacaggtttaaggagaccaatagaaactgggcttgtcgagacagagaagactcttgcgtttctgataggcacctattggtcttactgacatccactttgcctttctctccacaggtgtccactcccagttcaattacagctcttaaggctagagtacttaatacgactcactataggctagcctcgagaattcatggcttctagaatcctctggcatgagatgtggcatgaaggcctggaagaggcatctcgtttgtactttggggaaaggaacgtgaaaggcatgtttgaggtgctggagcccttgcatgctatgatggaacggggcccccagactctgaaggaaacatcctttaatcaggcctatggtcgagatttaatggaggcccaagagtggtgcaggaagtacatgaaatcagggaatgtcaaggacctcctccaagcctgggacctctattatcatgtgttccgacgaatctcaaagactagagatgagtttcccaccatggtgtttccttctgggcagatcagccaggcctcggccttggccccggcccctccccaagtcctgccccaggctccagcccctgcccctgctccagccatggtatcagctctggcccaggccccagcccctgtcccagtcctagccccaggccctcctcaggctgtggccccacctgcccccaagcccacccaggctggggaaggaacgctgtcagaggccctgctgcagctgcagtttgatgatgaagacctgggggccttgcttggcaacagcacagacccagctgtgttcacagacctggcatccgtcgacaactccgagtttcagcagctgctgaaccagggcatacctgtggccccccacacaactgagcccatgctgatggagtaccctgaggctataactcgcctagtgacaggggcccagaggccccccgacccagctcctgctccactgggggccccggggctccccaatggcctcctttcaggagatgaagacttctcctccattgcggacatggacttctcagccctgctgagtcagatcagctccactagttattaagaattcacgcgtcgagcatgcatctagggcggccaattccgcccctctcccccccccccctctccctcccccccccctaacgttactggccgaagccgcttggaataaggccggtgtgcgtttgtctatatgttattttccaccatattgccgtcttttggcaatgtgagggcccggaaacctggccctgtcttcttgacgagcattcctaggggtctttcccctctcgccaaaggaatgcaaggtctgttgaatgtcgtgaaggaagcagttcctctggaagcttcttgaagacaaacaacgtctgtagcgaccctttgcaggcagcggaaccccccacctggcgacaggtgcctctgcggccaaaagccacgtgtataagatacacctgcaaaggcggcacaaccccagtgccacgttgtgagttggatagttgtggaaagagtcaaatggctctcctcaagcgtattcaacaaggggctgaaggatgcccagaaggtaccccattgtatgggatctgatctggggcctcggtgcacatgctttacatgtgtttagtcgaggttaaaaaaacgtctaggccccccgaaccacggggacgtggttttcctttgaaaaacacgatgataagcttgccacaacccgggatcctctagagtcgacatggactatcctgctgccaagagggtcaagttggactctagagaacgcccatatgcttgccctgtcgagtcctgcgatcgccgcttttctcgctcggatgagcttacccgccatatccgcatccacacaggccagaagcccttccagtgtcgaatctgcatgcgtaacttcagtcgtagtgaccaccttaccacccacatccgcacccacacaggcggcggccgcaggaggaagaaacgcaccagcatagagaccaacatccgtgtggccttagagaagagtttcttggagaatcaaaagcctacctcggaagagatcactatgattgctgatcagctcaatatggaaaaagaggtgattcgtgtttggttctgtaaccgccgccagaaagaaaaaagaatcaacactagaggagtgcaggtggaaaccatctccccgggagacgggcgcaccttccccaagcgcggccagacctgcgtggtgcactacaccgggatgcttgaagatggaaagaaatttgattcctcccgggacagaaacaagccctttaagtttatgctaggcaagcaggaggtgatccgaggctgggaagaaggggttgcccagatgagtgtgggtcagagagccaaactgactatatctccagattatgcctatggtgccactgggcacccaggcatcatcccaccacatgccactctcgtcttcgatgtggagcttctaaaactggaagtcgagggcgtgcaggtggaaaccatctccccaggagacgggcgcaccttccccaagcgcggccagacctgcgtggtgcactacaccgggatgcttgaagatggaaagaaatttgattcctcccgggacagaaacaagccctttaagtttatgctaggcaagcaggaggtgatccgaggctgggaagaaggggttgcccagatgagtgtgggtcagagagccaaactgactatatctccagattatgcctatggtgccactgggcacccaggcatcatcccaccacatgccactctcgtcttcgatgtggagcttctaaaactggaaactagaggagtgcaggtggaaaccatctccccaggagacgggcgcaccttccccaagcgcggccagacctgcgtggtgcactacaccgggatgcttgaagatggaaagaaatttgattcctcccgggacagaaacaagccctttaagtttatgctaggcaagcaggaggtgatccgaggctgggaagaaggggttgcccagatgagtgtgggtcagagagccaaactgactatatctccagattatgcctatggtgccactgggcacccaggcatcatcccaccacatgccactctcgtcttcgatgtggagcttctaaaactggaaactagttattaagtcgacccgggcggccgcttccctttagtgagggttaatgcttcgagcagacatgataagatacattgatgagtttggacaaaccacaactagaatgcagtgaaaaaaatgctttatttgtgaaatttgtgatgctattgctttatttgtaaccattataagctgcaataaacaagttaacctccatagaagacaccgggaccgatccaataacttcgtatagcatacattatacgaagttatggctgctagtgaacyaatcwcatgatgtcacccagacatcaggcatacccactagtgtgaaatagacatcagaattaagaaaaatgggctccccgggcgcgtactccacctcacccatcatccacgctcggcaataaaaagacagaataaaacgcacgggtgttgggtcgtttgttcgttttatggatagcactgagaacgtcatcaagcccttcatgcgcttcaaggtgcacatggagggctccgtgaacggccacgagttcgagatcgagggcgagggcgagggcaagccctacgagggcacccagaccgccaagctgcaggtgaccaagggcggccccctgcccttcgcctgggacatcctgtccccccagttccagtacggctccaaggtgtacgtgaagcaccccgccgacatccccgactacaagaagctgtccttccccgagggcttcaagtgggagcgcgtgatgaacttcgaggacggcggcgtggtgaccgtgacccaggactcctccctgcaggacggcaccttcatctaccacgtgaagttcatcggcgtgaacttcccctccgacggccccgtaatgcagaagaagactctgggctgggagccctccaccgagcgcctgtacccccgcgacggcgtgctgaagggcgagatccacaaggcgctgaagctgaagggcggcggccactacctggtggagttcaagtcaatctacatggccaagaagcccgtgaagctgcccggctactactacgtggactccaagctggacatcacctcccacaacgaggactacaccgtggtggagcagtacgagcgcgccgaggcccgccaccacctgttccagtaggacctccatagaagacaccgaataaaatatctttattttcattacatctgtgtgttggttttttgtgtgaatcgatagtactaacatacgctctccatcaaaacaaaacgaaacaaaacaaactagcaaaataggctgtccccagtgcaagtgcaggtgccagaacatttctctggaccgatccaataacttcgtatagcatacattatacgaagttatgcctccggactctagcgttttagttattactagcgctaccggactcagatctcgagctcaagcttcgaattctgcagtcgacggtaccgcggcttacgcgtgctagctaatgatgggcgctcgagtaatgatgggcggtcgactaatgatgggcgctcgagtaatgatgggcgtctagctaatgatgggcgctcgagtaatgatgggcggtcgactaatgatgggcgctcgagtaatgatgggcgtctagctaatgatgggcgctcgagtaatgatgggcggtcgactaatgatgggcgctcgagtaatgatgggcgtctagaacgcgaattaattcaacattttgacacccccataatatttttccagaattaacagtataaattgcatctcttgttcaagagttccctatcactctctttaatcactactcacagtaacctcaactcctgccacaagcttgccctgcagcgggaattccaaacttaagcttggtaccgagctcggatccactagtccagtgtggtggaattctgcagatatccagcacagtggcggccgctcgagtctagagggcccgtttaaacccgctgatcagatggcaggaagaagcggagacagcgacgaagacctcctcaaggcagtcagactcatcaagtttctctatcaaagcaacccacctcccaaccccgaggggacccgacaggcccgaaggaatagaagaagaaggtggagagagagacagagacagatccattcgattagtgaacggatccttagcacttatttgggacgatctgcggacgctgtgcctcttcagctaccaccgcttgagagacttactcttgattgtgacgaggattgtggaacttctgggacgcagggggtgggaagccctcaaatattggtggaatctcctacaatattggagtcaggagctaaagaatagtccctcccccccccctaacgttactggccgaagccgcttggaataaggccggtgtgcgtttgtctatatgttattttccaccatattgccgtcttttggcaatgtgagggcccggaaacctggccctgtcttcttgacgagcattcctaggggtctttcccctctcgccaaaggaatgcaaggtctgttgaatgtcgtgaaggaagcagttcctctggaagcttcttgaagacaaacaacgtctgtagcgaccctttgcaggcagcggaaccccccacctggcgacaggtgcctctgcggccaaaagccacgtgtataagatacacctgcaaaggcggcacaaccccagtgccacgttgtgagttggatagttgtggaaagagtcaaatggctctcctcaagcgtattcaacaaggggctgaaggatgcccagaaggtaccccattgtatgggatctgatctggggcctcggtgcacatgctttacatgtgtttagtcgaggttaaaaaacgtctaggccccccgaaccacggggacgtggttttcctttgaaaaacacgatgataatggggaggaggaagaggaagccgaaggatccgaaggcgagggtgttggcggaggcggattacaaggacgacgatgacaagatgtcagatcccagggagagaatcccacctggaaacagtggagaagagacaataggagaggccttcgaatggctaaacagaacagtagaggagataaacagagaggcagtaaaccacctaccaagggagctgattttccaggtttggcaaaggtcttgggaatactggcatgatgaacaagggatgtcacaaagctatgtaaaatacagatacttgtgtttaatgcaaaaggctttatttatgcattgcaagaaaggctgtagatgtctaggggaaggacacggggcaggaggatggagaccaggacctcctcctcctccccctccaggactagcataacctcgactgtgccttctagttgccagccatctgttgtttgcccctcccccgtgccttccttgaccctggaaggtgccactcccactgtcctttcctaataaaatgaggaaattgcatcgcattgtctgagtaggtgtcattctattctggggggtggggtggggcaggacagcaagggggaggattgggaagacaatagcaggcatgctggggatgcggtgggctctatggcttctgaggcggaaagttaaccctagaaagataatcatattgtgacgtacgttaaagataatcatgcgtaaaattgacgcatgtgttttatcggtctgtatatcgaggtttatttattaatttgaatagatattaagttttattatatttacacttacatactaataataaattcaacaaacaatttatttatgtttatttatttattaaaaaaaaacaaaaactcaaaatttcttctataaagtaacaaaaaccagctggggctcgaagttcctatactttctagagaataggaacttctatagtgagtcgaataagggcgacacaaaatttattctaaatgcataataaatactgataacatcttatagtttgtattatattttgtattatcgttgacatgtataattttgatatcaaaaactgattttccctttattattttcgagatttattttcttaattctctttaacaaactagaaatattgtatatacaaaaaatcataaataatagatgaatagtttaattataggtgttcatcaatcgaaaaagcaacgtatcttatttaaagtgcgttgcttttttctcatttataaggttaaataattctcatatatcaagcaaagtgacaggcgcccttaaatattctgacaaatgctctttccctaaactccccccataaaaaaacccgccgaagcgggtttttacgttatttgcggattaacgattactcgttatcagaaccgcccagggggcccgagcttaagactggccgtcgttttacaacacagaaagagtttgtagaaacgcaaaaaggccatccgtcaggggccttctgcttagtttgatgcctggcagttccctactctcgccttccgcttcctcgctcactgactcgctgcgctcggtcgttcggctgcggcgagcggtatcagctcactcaaaggcggtaatacggttatccacagaatcaggggataacgcaggaaagaacatgtgagcaaaaggccagcaaaaggccaggaaccgtaaaaaggccgcgttgctggcgtttttccataggctccgcccccctgacgagcatcacaaaaatcgacgctcaagtcagaggtggcgaaacccgacaggactataaagataccaggcgtttccccctggaagctccctcgtgcgctctcctgttccgaccctgccgcttaccggatacctgtccgcctttctcccttcgggaagcgtggcgctttctcatagctcacgctgtaggtatctcagttcggtgtaggtcgttcgctccaagctgggctgtgtgcacgaaccccccgttcagcccgaccgctgcgccttatccggtaactatcgtcttgagtccaacccggtaagacacgacttatcgccactggcagcagccactggtaacaggattagcagagcgaggtatgtaggcggtgctacagagttcttgaagtggtgggctaactacggctacactagaagaacagtatttggtatctgcgctctgctgaagccagttaccttcggaaaaagagttggtagctcttgatccggcaaacaaaccaccgctggtagcggtggtttttttgtttgcaagcagcagattacgcgcagaaaaaaaggatctcaagaagatcctttgatcttttctacggggtctgacgctcagtggaacgacgcgcgcgtaactcacgttaagggattttggtcatgagcttgcgccgtcccgtcaagtcagcgtaatgctctgcttttagaaaaactcatcgagcatcaaatgaaactgcaatttattcatatcaggattatcaataccatatttttgaaaaagccgtttctgtaatgaaggagaaaactcaccgaggcagttccataggatggcaagatcctggtatcggtctgcgattccgactcgtccaacatcaatacaacctattaatttcccctcgtcaaaaataaggttatcaagtgagaaatcaccatgagtgacgactgaatccggtgagaatggcaaaagtttatgcatttctttccagacttgttcaacaggccagccattacgctcgtcatcaaaatcactcgcatcaaccaaaccgttattcattcgtgattgcgcctgagcgaggcgaaatacgcgatcgctgttaaaaggacaattacaaacaggaatcgagtgcaaccggcgcaggaacactgccagcgcatcaacaatattttcacctgaatcaggatattcttctaatacctggaacgctgtttttccggggatcgcagtggtgagtaaccatgcatcatcaggagtacggataaaatgcttgatggtcggaagtggcataaattccgtcagccagtttagtctgaccatctcatctgtaacatcattggcaacgctacctttgccatgtttcagaaacaactctggcgcatcgggcttcccatacaagcgatagattgtcgcacctgattgcccgacattatcgcgagcccatttatacccatataaatcagcatccatgttggaatttaatcgcggcctcgacgtttcccgttgaatatggctcatattcttcctttttcaatattattgaagcatttatcagggttattgtctcatgagcggatacatatttgaatgtatttagaaaaataaacaaataggggtcagtgttacaaccaattaaccaattctgaacattatcgcgagcccatttatacctgaatatggctcataacaccccttgtttgcctggcggcagtagcgcggtggtcccacctgaccccatgccgaactcagaagtgaaacgccgtagcgccgatggtagtgtggggactccccatgcgagagtagggaactgccaggcatcaaataaaacgaaaggctcagtcgaaagactgggcctttcgcccgggctaattagggggtgtcgcccttattcgactctatagtgaagttcctattctctagaaagtataggaacttctgaagt

SEQ ID NO: 87 - RNA, 76 nt, Artificial sequence
  synthetic Evolved aptamer
gggcggcacuuauacagcgaagcauaauggcuacugacgcccucaaacccuauuugcagacuauaagugucgcgcg

SEQ ID NO: 88 - RNA, 73 nt, Artificial sequence
  synthetic Evolved aptamer
gggcggcacuuauacaggguagcauaauggcuuaggacgccuucaaaccuaucaagacuauaagugucgcgcg

SEQ ID NO: 89 - RNA, 75 nt, Artificial sequence
  synthetic Evolved aptamer
gggcggcacuuauacaggguagcauaaugggcuacuugacgccuucaccuauuuguagacuauaagugucgcgcg

SEQ ID NO: 90 - RNA, 76 nt, Artificial sequence
  synthetic Evolved aptamer
gggcggcacuuauacagcguagcauaaugggcugcagacgccgucaaaccuauuugcagacuauaagugucgcgcg

SEQ ID NO: 91 - RNA, 74 nt, Artificial sequence
  synthetic Evolved aptamer
gggcggcacuuauacaccguagcauaaugggcuacugccgccgucgaccuuuuggagacuauaagugucgcgcg

SEQ ID NO: 92 - RNA, 75 nt, Artificial sequence
  synthetic Evolved aptamer
gggcggcacuuauacaggucagcauaaugugcuagugcgccuucaaaccuauuuagagacuauaagugucgcgcg

SEQ ID NO: 93 - RNA, 76 nt, Artificial sequence
  synthetic Evolved aptamer
gggcggcacuuauacagcuuagcguaauggcuacugacgccguccaaaccuauuuacagacuauaagugucgcgcg

SEQ ID NO: 94 - RNA, 76 nt, Artificial sequence
  synthetic Evolved aptamer
gggcggcacuuauacaggggagcauaaugggcuacugacgccuuuaaaccuauuugaggacuauaagugucgcgcg

SEQ ID NO: 95 - RNA, 74 nt, Artificial sequence
  synthetic Evolved aptamer
gggcggcacuuauacauggaagcauaaugggcugccgacggcccuuaaccuuuggagacuauaagugucgcgcg

SEQ ID NO: 96 - RNA, 79 nt, Artificial sequence
  synthetic Evolved aptamer
gggcggcacuuauacagauuagcauaaugggcuacugaccccgccggcaaaccuauuugaagacuauaagugucgcgcg

SEQ ID NO: 97 - RNA, 75 nt, Artificial sequence
  synthetic Evolved aptamer
gggcggcacuuauacaguguagcauaaugggcuacugucgcaucaaaccuauuuggagacuauaagugucgcgcg

SEQ ID NO: 98 - RNA, 76 nt, Artificial sequence
  synthetic Evolved aptamer
gggcggcacuuauacagugaagcauaaugggcuacugacacccuuaaaccuauuugcagacuauaagugucgcgcg

SEQ ID NO: 99 - RNA, 76 nt, Artificial sequence
  synthetic Evolved aptamer
gggcggcacuuauacagaguagcauaaugggcuacagacgccgucaaaccuauuuaccgacuauaagugucgcgcg

SEQ ID NO: 100 - RNA, 75 nt, Artificial sequence
  synthetic Evolved aptamer
gggcggcacuuauacagggugcauaaugggcuagugacgccuucaaaccuauuuguagacuauaagugucgcgcg

SEQ ID NO: 101 - protein, 461 aa, Homo sapiens
MTILGTTFGMVFSLLQVVSGESGYAQNGDLEDAELDDYSFSCYSQLEVNGSQHSLTCAFEDPDVNTTNLEFEICGALVEVKCLNFRKLQEIYFIETKKFLLIGKSNICVKVGEKSLTCKKIDLTTIVKPEAPFDLSVIYREGANDFVVTFNTSHLQKKYVKVLMHDVAYRQEKDENKWTHVNLSSTKLTLLQRKLQPAAMYEIKVRSIPDHYFKGFWSEWSPSYYFRTPEINNSSGEMDPILLTISKCHLSFFSVALLVILACVLWKKRIKPIVWPSLPDHKKTLEHLCKKPRKNLNVSFNPESFLDCQIHRVDDIQARDEVEGFLQDTFPQQLEESEKQRLGGDVQSPNCPSEDVVVTPESFGRDSSLTCLAGNVSACDAPILSSSRSLDCRESGKNGPHVYQDLLLSLGTTNSTLPPPFSLQSGILTLNPVAQGQPILTSLGSNQEEAYVTMSSFYQNQ

SEQ ID NO: 102 - protein, 463 aa, Homo sapiens
MTILGTTFGMVFSLLQVVSGESGYAQNGDLEDAELDDYSFSCYSQLEVNGSQHSLTCAFEDPDVNTTNLEFEICGALVEVKCLNFRKLQEIYFIETKKFLLIGKSNICVKVGEKSLTCKKIDLTTIVKPEAPFDLSVIYREGANDFVVTFNTSHLQKKYVKVLMHDVAYRQEKDENKWTHVNLSSTKLTLLQRKLQPAAMYEIKVRSIPDHYFKGFWSEWSPSYYFRTPEINNSSGEMDPIFSCGPLTISILSFFSVALLVILACVLWKKRIKPIVWPSLPDHKKTLEHLCKKPRKNLNVSFNPESFLDCQIHRVDDIQARDEVEGFLQDTFPQQLEESEKQRLGGDVQSPNCPSEDVVVTPESFGRDSSLTCLAGNVSACDAPILSSSRSLDCRESGKNGPHVYQDLLLSLGTTNSTLPPPFSLQSGILTLNPVAQGQPILTSLGSNQEEAYVTMSSFYQNQ

SEQ ID NO: 103 - protein, 462 aa, Homo sapiens
MTILGTTFGMVFSLLQVVSGESGYAQNGDLEDAELDDYSFSCYSQLEVNGSQHSLTCAFEDPDVNTTNLEFEICGALVEVKCLNFRKLQEIYFIETKKFLLIGKSNICVKVGEKSLTCKKIDLTTIVKPEAPFDLSVIYREGANDFVVTFNTSHLQKKYVKVLMHDVAYRQEKDENKWTHVNLSSTKLTLLQRKLQPAAMYEIKVRSIPDHYFKGFWSEWSPSYYFRTPEINNSSGEMDPILLTCHLISILSFFSVALLVILACVLWKKRIKPIVWPSLPDHKKTLEHLCKKPRKNLNVSFNPESFLDCQIHRVDDIQARDEVEGFLQDTFPQQLEESEKQRLGGDVQSPNCPSEDVVVTPESFGRDSSLTCLAGNVSACDAPILSSSRSLDCRESGKNGPHVYQDLLLSLGTTNSTLPPPFSLQSGILTLNPVAQGQPILTSLGSNQEEAYVTMSSFYQNQ

SEQ ID NO: 104 - protein, 466 aa, Homo sapiens
MTILGTTFGMVFSLLQVVSGESGYAQNGDLEDAELDDYSFSCYSQLEVNGSQHSLTCAFEDPDVNTTNLEFEICGALVEVKCLNFRKLQEIYFIETKKFLLIGKSNICVKVGEKSLTCKKIDLTTIVKPEAPFDLSVIYREGANDFVVTFNTSHLQKKYVKVLMHDVAYRQEKDENKWTHVNLSSTKLTLLQRKLQPAAMYEIKVRSIPDHYFKGFWSEWSPSYYFRTPEINNSSGEMDPILLTPPVCSVTISILSFFSVALLVILACVLWKKRIKPIVWPSLPDHKKTLEHLCKKPRKNLNVSFNPESFLDCQIHRVDDIQARDEVEGFLQDTFPQQLEESEKQRLGGDVQSPNCPSEDVVVTPESFGRDSSLTCLAGNVSACDAPILSSSRSLDCRESGKNGPHVYQDLLLSLGTTNSTLPPPFSLQSGILTLNPVAQGQPILTSLGSNQEEAYVTMSSFYQNQ

SEQ ID NO: 105 - protein, 523 aa, Artificial sequence
  synthetic Fc-delta-30
MSIMGLKVNVSAIFMAVLLTLQTPTGQIHWGNLSKIGVVGIGSASYKVMTRSSHQSLVIKLMPNITLLNNCTRVEIAEYRRLLRTVLEPIRDALNAMTQNIRPVQSVASSRRHKRFAGVVLAGAALGVATAAQITAGIALHQSMLNSQAIDNLRASLETTNQAIEAIRQAGQEMILAVQGVQDYINNELIPSMNQLSCDLIGQKLGLKLLRYYTEILSLFGPSLRDPISAEISIQALSYALGGDINKVLEKLGYSGGDLLGILESRGIKARITHVDTESYFIVLSIAYPTLSEIKGVIVHRLEGVSYNIGSQEWYTTVPKYVATQGYLISNFDESSCTFMPEGTVCSQNALYPMSPLLQECLRGSTKSCARTLVSGSFGNRFILSQGNLIANCASILCKCYTTGTIINQDPDKILTYIAADHCPVVEVNGVTIQVGSRRYPDAVYLHRIDLGPPISLERLDVGTNLGNAIAKLEDAKELLESSDQILRSMKGLSSTSIVYILIAVCLGGLIGIPALICCCRGR

SEQ ID NO: 106 - protein, 599 aa, Artificial sequence
  synthetic Hc-delta-18
MGSRIVINREHLMIDRPYVLLAVLFVMSLSLIGLLAIAGIRLHRAAIYTAEIHKSLSTNLDVTNSIEHQVKDVLTPLFKIIGDEVGLRTPQRFTDLVKFISDKIKFLNPDREYDFRDLTWCINPPERIKLDYDQYCADVAAEELMNALVNSTLLETRTTNQFLAVSKGNCSGPTTIRGQFSNMSLSLLDLYLSRGYNVSSIVTMTSQGMYGGTYLVEKPNLSSKRSELSQLSMYRVFEVGVIRNPGLGAPVFHMTNYLEQPVSNDLSNCMVALGELKLAALCHGEDSITIPYQGSGKGVSFQLVKLGVWKSPTDMQSWVPLSTDDPVIDRLYLSSHRGVIADNQAKWAVPTTRTDDKLRMETCFQQACKGKIQALCENPEWAPLKDNRIPSYGVLSVDLSLTVELKIKIASGFGPLITHGSGMDLYKSNHNNVYWLTIPPMKNLALGVINTLEWIPRFKVSPNLFTVPIKEAGEDCHAPTYLPAEVDGDVKLSSNLVILPGQDLQYVLATYDTSRVEHAVVYYVYSPGRSFSYFYPFRLPIKGVPIELQVECFTWDQKLWCRHFCVLADSESGGHITHSGMVGMGVSCTVTREDGTNRR

SEQ ID NO: 107 - protein, 529 aa, Artificial sequence
  synthetic DAFss-IL7-DAF fusion
MTVARPSVPAALPLLGELPRLLLLVLLCLPADCDIEGKDGKQYESVLMVSIDQLLDSMKEIGSNCLNNEFNFFKRHICDANKEGMFLFRAARKLRQFLKMNSTGDFDLHLLKVSEGTTILLNCTGQVKGRKPAALGEAQPTKSLEENKSLKEQKKLNDLCFLKRLLQEIKTCWNKILMGTKEHCGLPPDVPNAQPALEGRTSFPEDTVITYKCEESFVKIPGEKDSVICLKGSQWSDIEEFCNRSCEVPTRLNSASLKQPYITQNYFPVGTVVEYECRPGYRREPSLSPKLTCLQNLKWSTAVEFCKKKSCPNPGEIRNGQIDVPGGILFGATISFSCNTGYKLFGSTSSFCLISGSSVQWSDPLPECREIYCPAPPQIDNGIIQGERDHYGYRQSVTYACNKGFTMIGEHSIYCTVNNDEGEWSGPPPECRGKSLTSKVPPTVQKPTTVNVPTTEVSPTSQKTTTKTTTPNAQATRSTPVSRTTKHFHETTPNKGSGTTSGTTRLLSGHTCFTLTGLLGTLVTMGLLT

SEQ ID NO: 108 - DNA, 49 bp, Artificial sequence
  synthetic 582-1
acagcttagcgtaatggctactgacgccgtccaaacctatttacagact

SEQ ID NO: 109 - DNA, 49 bp, Artificial sequence
  synthetic 582-2
acagcttaggataatggctactgacgccgtccaaacctatttacagact

SEQ ID NO: 110 - DNA, 49 bp, Artificial sequence
  synthetic 582-3
acagcttagcataatggctactgacgccgtccaaacctattcacagact

SEQ ID NO: 111 - DNA, 49 bp, Artificial sequence
  synthetic 582-4
acagcttagcataatggctactgacgccgtccaaacctattgacagact

SEQ ID NO: 112 - DNA, 49 bp, Artificial sequence
  synthetic 582-5
acagcatagcataatggctactgacgccgtccaaacctatttacagact

SEQ ID NO: 113 - DNA, 49 bp, Artificial sequence
  synthetic 582-6
acagcttagcataatggctactgacgccgtccaaacctatgtacagact

SEQ ID NO: 114 - DNA, 48 bp, Artificial sequence
  synthetic 582-7
acagctagcgtaatggctactgacgccgtccaaacctatttacagact

SEQ ID NO: 115 - DNA, 49 bp, Artificial sequence
  synthetic 582-8
acagcttagcattatggctactgacgccgtccaaacctatttacagact

SEQ ID NO: 116 - DNA, 48 bp, Artificial sequence
  synthetic 582-9
acagttagcataatggctactgacgccgtccaaacctatttacagact

SEQ ID NO: 117 - DNA, 49 bp, Artificial sequence
  synthetic 582-10
acagcttagcataatggctactgacgcggtccaaacctatttacagact

SEQ ID NO: 118 - DNA, 49 bp, Artificial sequence
  synthetic 582-11
acagcttagcttaatggctactgacgccgtccaaacctatttacagact

SEQ ID NO: 119 - DNA, 49 bp, Artificial sequence
  synthetic 582-12
acagcttagcataatggctactgacgccgtccaaacccatttacagact

SEQ ID NO: 120 - DNA, 49 bp, Artificial sequence
  synthetic 582-13
acagcttagcataatggctactgacgccgtccaaaccaatttacagact

SEQ ID NO: 121 - DNA, 49 bp, Artificial sequence
  synthetic 582-14
acagcttagcataatggatactgacgccgtccaaacctatttacagact

SEQ ID NO: 122 - DNA, 49 bp, Artificial sequence
  synthetic 582-15
acagcttagcattgtggctactgacgccgtccaaacctatttacagact

SEQ ID NO: 123 - DNA, 49 bp, Artificial sequence
  synthetic 582-16
acaggttagcataatggctaccgacgccgtccaaacctatttacagact

SEQ ID NO: 124 - DNA, 49 bp, Artificial sequence
  synthetic 582-17
acagcttagcgtaatggctactgacgccgcccaaacctatttacagact

SEQ ID NO: 125 - DNA, 49 bp, Artificial sequence
  synthetic 582-18
acagcttagcataatggctactgacgccgtccaaaactatttccagact

SEQ ID NO: 126 - DNA, 49 bp, Artificial sequence
  synthetic 582-19
acagcctagcataagggctactgacgccgtccaaacctatttacagact

SEQ ID NO: 127 - DNA, 49 bp, Artificial sequence
  synthetic 582-20
acagcttagcataatggctactgaggccgtccaaacctatttacagact

SEQ ID NO: 128 - DNA, 49 bp, Artificial sequence
  synthetic 582-21
acagcttaccttaatggctactgacgccgtccaaacctatttacagact

SEQ ID NO: 129 - DNA, 49 bp, Artificial sequence
  synthetic 582-22
acagcttagcataatggctaccgacgctgtccaaacctatttacagact

SEQ ID NO: 130 - DNA, 49 bp, Artificial sequence
  synthetic 582-23
acagcttagcgtaatggctactggcgccgtccaaacctatttacagact

SEQ ID NO: 131 - DNA, 49 bp, Artificial sequence
  synthetic 582-24
acagcttagcatactggctactgacgccgcccaaacctatttacagact

SEQ ID NO: 132 - DNA, 49 bp, Artificial sequence
  synthetic 582-25
acagcttagcataatggctactgacgccgtcctaacctatttacagact

SEQ ID NO: 133 - DNA, 49 bp, Artificial sequence
  synthetic 582-26
acaggttagcataatgcctactgacgccgtccaaacctatttacagact

SEQ ID NO: 134 - DNA, 49 bp, Artificial sequence
  synthetic 582-27
acagcttagcataattgctactgacgccgttcaaacctatttacagact

SEQ ID NO: 135 - DNA, 49 bp, Artificial sequence
  synthetic 582-28
acagcttagcataaaggctactgacgccgtccaaacctatttacagact

SEQ ID NO: 136 - DNA, 49 bp, Artificial sequence
  synthetic 582-29
acagcttagcgtaatggctactgacgccgtctaaacctatttccagact

SEQ ID NO: 137 - DNA, 49 bp, Artificial sequence
  synthetic 582-30
acaggttagcataatggctactgacgccgtccaaacctatttagagact

SEQ ID NO: 138 - DNA, 49 bp, Artificial sequence
  synthetic 582-31
acagggtagcgtaatggctactgacgccgtccaaacctatttacagact

SEQ ID NO: 139 - DNA, 49 bp, Artificial sequence
  synthetic 582-32
acagcgtagcataatggctactgacgccgttcaaacctatttacagact

SEQ ID NO: 140 - DNA, 49 bp, Artificial sequence
  synthetic 582-33
acagcttagcataatggctactgacgccgtccaaactcatttacagact

SEQ ID NO: 141 - DNA, 49 bp, Artificial sequence
  synthetic 582-34
acagcgtagcatagtggctactgacgccgtccaaacctatttacagact

SEQ ID NO: 142 - DNA, 49 bp, Artificial sequence
  synthetic 582-35
acagcttagtgtaatggctactgacgctgtccaaacctatttacagact

SEQ ID NO: 143 - DNA, 49 bp, Artificial sequence
  synthetic 582-36
acagcttagcataatggctactgacggcgttcaaacctatttacagact

SEQ ID NO: 144 - DNA, 49 bp, Artificial sequence
  synthetic 582-37
acaggttagcataatggctactgacgccgtccaaacctatttatagact

SEQ ID NO: 145 - DNA, 48 bp, Artificial sequence
  synthetic 582-38
acagcttagcataatggctactgacgccgtccaaacctattgtcgact

SEQ ID NO: 146 - DNA, 48 bp, Artificial sequence
  synthetic 582-39
acagcttagcataatggctactgacgccgtccaaacctatttacgact

SEQ ID NO: 147 - DNA, 48 bp, Artificial sequence
  synthetic 769-1
acaggtcagcataatgtgctagtgcgccttcaaacctatttagagact

SEQ ID NO: 148 - DNA, 48 bp, Artificial sequence
  synthetic 769-2
acaggtcagcataatgtgctagtgcgccctcaaacctatttagagact

SEQ ID NO: 149 - DNA, 48 bp, Artificial sequence
  synthetic 769-3
acaggttagcataatgtgctattgcgccttcaaacctatttagagact

SEQ ID NO: 150 - DNA, 48 bp, Artificial sequence
  synthetic 769-4
acaggtcagcataatgtgctagtgcgcattcaaacctatttagagact

SEQ ID NO: 151 - DNA, 48 bp, Artificial sequence
  synthetic 769-5
acaggttagcataatgtgctagtgcgccttcaaacctattttgagact

SEQ ID NO: 152 - DNA, 48 bp, Artificial sequence
  synthetic 769-6
acaggttatcataatgtgctagtgcgccttcaaacctatttagagact

SEQ ID NO: 153 - DNA, 48 bp, Artificial sequence
  synthetic 769-7
acaggttagcatgatgtgctagtgcgccttcaaacctatttagagact

SEQ ID NO: 154 - DNA, 48 bp, Artificial sequence
  synthetic 769-8
acaggttagcataatgggctagtgcgccttcaaacctatttagagact

SEQ ID NO: 155 - DNA, 48 bp, Artificial sequence
  synthetic 769-9
acaggtcagcaaaatgtgcaagtgcgccttcaaacctatttagagact

SEQ ID NO: 156 - DNA, 48 bp, Artificial sequence
  synthetic 769-10
acaggtcagcataatgtgctagtgcgccttcaaacctatctggagact

SEQ ID NO: 157 - DNA, 48 bp, Artificial sequence
  synthetic 769-11
acagcttagcataatgtgctagtgcgccttcaaacctatttagagact

SEQ ID NO: 158 - DNA, 48 bp, Artificial sequence
  synthetic 769-12
acaggtcagcataatgtgctagtgcgccttcaaacctatttacagact

SEQ ID NO: 159 - DNA, 48 bp, Artificial sequence
  synthetic 769-13
acaggtcagcataatgtgctagtgcgccttcaaacatatttagagact

SEQ ID NO: 160 - DNA, 48 bp, Artificial sequence
  synthetic 769-14
acagggtagcataatgtgctagtgcgccttcaaacctatttagagact

SEQ ID NO: 161 - DNA, 48 bp, Artificial sequence
  synthetic 769-15
acaggttagcataatgtgctagtgcgccctcaaacctatttagagact

SEQ ID NO: 162 - DNA, 48 bp, Artificial sequence
  synthetic 769-16
acaggttagcataatgtgccagtgcgccttcaaacctatttagagact

SEQ ID NO: 163 - DNA, 48 bp, Artificial sequence
  synthetic 769-17
acaggtcagcataatgggctagtgcgccttcaaacctatttagagact

SEQ ID NO: 164 - DNA, 49 bp, Artificial sequence
  synthetic 795-1
acagcgaagcataatggctactgacgccctcaaaccctatttgcagact

SEQ ID NO: 165 - DNA, 49 bp, Artificial sequence
  synthetic 795-2
acagcgaagcataatggctactgacgccctcaaaccctatttacagact

SEQ ID NO: 166 - DNA, 49 bp, Artificial sequence
  synthetic 795-3
acagcgaagcataatggcttctgacgccctcaaaccctatttgcagact

SEQ ID NO: 167 - DNA, 49 bp, Artificial sequence
  synthetic 795-4
acagccaagcatactggctactgacgccctcaaaccctatttgcagact

SEQ ID NO: 168 - DNA, 49 bp, Artificial sequence
  synthetic 795-5
acagcgaagcataatggctactgacgcccgcaaaccctatttgcagact

SEQ ID NO: 169 - DNA, 49 bp, Artificial sequence
  synthetic 795-6
acagcgaagcataatggctactgacggcctcaaaccctatttgcagact

SEQ ID NO: 170 - DNA, 49 bp, Artificial sequence
  synthetic 795-7
acagcgaggcataatggctactgacgccctcaaaccctatttgcagact

SEQ ID NO: 171 - DNA, 49 bp, Artificial sequence
  synthetic 795-8
acagcgaagcataatggctactgacgccttcaaaccctatttgcagact

SEQ ID NO: 172 - DNA, 49 bp, Artificial sequence
  synthetic 795-9
acagcgaagcataatggctacagacgccctcaaaacctatttgcagact

SEQ ID NO: 173 - DNA, 48 bp, Artificial sequence
  synthetic 795-10
acagcgaagcataatggctactgacgccctcaaaccctatttgagact

SEQ ID NO: 174 - DNA, 48 bp, Artificial sequence
  synthetic 795-11
acagcgaagcataatggctactgacgccctcaaaccctattgtcgact

SEQ ID NO: 175 - DNA, 49 bp, Artificial sequence
  synthetic 795-12
acagccaagcataatggctactgacgccctcaaaccctatttgcagact

SEQ ID NO: 176 - DNA, 49 bp, Artificial sequence
  synthetic 795-13
acagcgaagcataatggctactgacgccctcaaaccctatttggcgact

SEQ ID NO: 177 - DNA, 49 bp, Artificial sequence
  synthetic 795-14
acagcgaagcataatgtctactgacgccctcaaaccctatttgcagact

SEQ ID NO: 178 - DNA, 49 bp, Artificial sequence
  synthetic 795-15
acagcgaagcataatggctactgacgccgtcaaaccctatttgtagact

SEQ ID NO: 179 - DNA, 49 bp, Artificial sequence
  synthetic 795-16
acagcgaagcataatggctactgacgccctcaaaccttatttgcagact

SEQ ID NO: 180 - DNA, 48 bp, Artificial sequence
  synthetic 795-17
acaggtagcataatggctactgacgccctcaaaccctatttgcagact

SEQ ID NO: 181 - DNA, 49 bp, Artificial sequence
  synthetic 795-18
acagcgaagcataatggctactgacgccctcaaaccctatttctagact

SEQ ID NO: 182 - DNA, 49 bp, Artificial sequence
  synthetic 795-19
acagcgaagcataatggctactgacgccctcaaaccctatttgtagact

SEQ ID NO: 183 - DNA, 48 bp, Artificial sequence
  synthetic 935-1
acagggtagcataatgggctacttgacgccttcacctatttgtagact

SEQ ID NO: 184 - DNA, 47 bp, Artificial sequence
  synthetic 935-2
acagggtagcataatgggctacttgacgccttcacctatttgagact

SEQ ID NO: 185 - DNA, 48 bp, Artificial sequence
  synthetic 935-3
acagggtagcataatgggctactttacgccttcacctatttgtagact

SEQ ID NO: 186 - DNA, 48 bp, Artificial sequence
  synthetic 935-4
acagggtagcataatgggctacttgacgccttcacctatttctagact

SEQ ID NO: 187 - DNA, 48 bp, Artificial sequence
  synthetic 935-5
acagggtagcataatgggctacttgacgccttcacctatttggagact

SEQ ID NO: 188 - DNA, 48 bp, Artificial sequence
  synthetic 935-6
acagggtagcatagtgggctacttgacgccttcacctatttgtagact

SEQ ID NO: 189 - DNA, 48 bp, Artificial sequence
  synthetic 935-7
acagggtagcatgatgggctacttgacgccttcacctatttgtagact

SEQ ID NO: 190 - DNA, 48 bp, Artificial sequence
  synthetic 935-8
acagggtagcataatgggctacttgacgccttcacctattagtagact

SEQ ID NO: 191 - DNA, 48 bp, Artificial sequence
  synthetic 935-9
acagggtagcataatgggctatttgacgccttcacctatttgtagact

SEQ ID NO: 192 - DNA, 48 bp, Artificial sequence
  synthetic 935-10
acagggtagcataatgggctacttgccgccttcacctatttgtagact

SEQ ID NO: 193 - DNA, 48 bp, Artificial sequence
  synthetic 935-11
acagtgtagcataattggctacttgacgccttcacctatttgtagact

SEQ ID NO: 194 - DNA, 48 bp, Artificial sequence
  synthetic 935-12
acagggtagcataatgggctacttgacgctttcacctttttgtagact

SEQ ID NO: 195 - DNA, 48 bp, Artificial sequence
  synthetic 935-13
acagggtagcataaggggctacttgacgccttcacctatttgtagact

SEQ ID NO: 196 - DNA, 48 bp, Artificial sequence
  synthetic 935-14
acagggtagcataatggactacttgacgcctccacctatttgtagact

SEQ ID NO: 197 - DNA, 48 bp, Artificial sequence
  synthetic 935-15
acagggtagcataatgggctacttgtcgccttcacctatttgtagact

SEQ ID NO: 198 - DNA, 49 bp, Artificial sequence
  synthetic 946-1
acagcgtagcataatgggctgcagacgccgtcaaacctatttgcagact

SEQ ID NO: 199 - DNA, 49 bp, Artificial sequence
  synthetic 946-2
acagcgtagcataatgggctgcagacgcagtcaaacctatttgcagact

SEQ ID NO: 200 - DNA, 48 bp, Artificial sequence
  synthetic 946-3
acatgtagcataatgggctactgacgccgtcaaacctatttgcagact

SEQ ID NO: 201 - DNA, 49 bp, Artificial sequence
  synthetic 946-4
acagcgtagcatagtgggctgcagacgccgtcaaacctatttgcagact

SEQ ID NO: 202 - DNA, 49 bp, Artificial sequence
  synthetic 946-5
acagtgtagcataatgggctgcagacgccttcaaacctatttggagact

SEQ ID NO: 203 - DNA, 49 bp, Artificial sequence
  synthetic 946-6
acagtgtagcataatgggctgctgacgccgtcaaacctatttgaagact

SEQ ID NO: 204 - DNA, 49 bp, Artificial sequence
  synthetic 946-7
acagcgtagcataatgggctacaggcgccgtcaaacctatttgcagact

SEQ ID NO: 205 - DNA, 49 bp, Artificial sequence
  synthetic 946-8
acagcgtagcataatgggctactggcgccgtcaaacctatttgcagact

SEQ ID NO: 206 - DNA, 48 bp, Artificial sequence
  synthetic 946-9
acagcgtagcataatgggctgcagacgccgtcaaacctatttgagact

SEQ ID NO: 207 - DNA, 48 bp, Artificial sequence
  synthetic 946-10
acaggtagcataatgggctgcagacgccgtcaaacctatttgcagact

SEQ ID NO: 208 - DNA, 48 bp, Artificial sequence
  synthetic 946-11
acaggtagcataatgggctgctgacgccgtcaaacctatttacagact

SEQ ID NO: 209 - DNA, 49 bp, Artificial sequence
  synthetic 946-12
acagcgtagcatattgggctgcagacgccgtcaaacctatttgcagact

SEQ ID NO: 210 - DNA, 49 bp, Artificial sequence
  synthetic 946-13
acagcgtagcataatgggctgcagacgccttcaaacctatttggagact

SEQ ID NO: 211 - DNA, 48 bp, Artificial sequence
  synthetic 946-14
acagtgtagcataatgggctgcagacgccgtcaaacctatttgagact

SEQ ID NO: 212 - DNA, 49 bp, Artificial sequence
  synthetic 946-15
acagcgtagcataatgggctgctgacgccgtcaaacctatttggagact

SEQ ID NO: 213 - DNA, 49 bp, Artificial sequence
  synthetic 946-16
acagcgtagcataatgggctgcagacgccgtcaaacctatttacagact

SEQ ID NO: 214 - DNA, 49 bp, Artificial sequence
  synthetic 946-17
acagcgtagcataatgggctgctgacgccgtcaaacctatttgcagact

SEQ ID NO: 215 - DNA, 49 bp, Artificial sequence
  synthetic 946-18
acagggtagcataatgggctgcagacgccgtcaaacctatttggagact

SEQ ID NO: 216 - DNA, 49 bp, Artificial sequence
  synthetic 946-19
acagcgtagcataatgggctacagacgccgtcaaacctatttgcagact

SEQ ID NO: 217 - DNA, 49 bp, Artificial sequence
  synthetic 946-20
acagcgtcgcataatgggctgcagacgccgtcaaatctatttgcagact

SEQ ID NO: 218 - DNA, 49 bp, Artificial sequence
  synthetic 946-21
acagcgtagcataatgggcttcagacgccgtcaaacctatttgcagact

SEQ ID NO: 219 - DNA, 48 bp, Artificial sequence
  synthetic 946-22
acatgtagcataatgggctgcagacgccgtcaaacctatttggagact

SEQ ID NO: 220 - DNA, 47 bp, Artificial sequence
  synthetic 961-1
acaccgtagcataatgggctactgccgccgtcgaccttttggagact

SEQ ID NO: 221 - DNA, 46 bp, Artificial sequence
  synthetic 996-1
acagggtagcataatggcttaggacgccttcaaacctatcaagact

SEQ ID NO: 222 - DNA, 49 bp, Artificial sequence
  synthetic Family 582 Consensus
  misc_feature (5)..(5): n at position 5 can be C, G, or no nucleotide
  misc_feature (6)..(6): n at position 6 can be A, C, G, T, or no nucleotide
  misc_feature (45)..(45): n at position 45 can be A or no nucleotide
acagnntasbdtwvdksmtacygrsgsbgyyywaamyhatkbhbngact

SEQ ID NO: 223 - DNA, 48 bp, Artificial sequence
  synthetic Family 769 Consensus
acagskyakcawratgkgchaktgcgcmytcaaacmtatytdsagact

SEQ ID NO: 224 - DNA, 49 bp, Artificial sequence
  synthetic Family 795 Consensus
  misc_feature (5)..(5): n at position 5 can be C or no nucleotide
  misc_feature (40)..(40): n at position 40 can be T or no nucleotide
  misc_feature (44)..(44): n at position 44 can be C, G, T, or no nucleotide
acagnswrgcatamtgkctwcwgacgscbkcaaamcytanttvnmgact

SEQ ID NO: 225 - DNA, 48 bp, Artificial sequence
  synthetic Family 935 Consensus
  misc_feature (43)..(43): n at position 43 can be G, T, or no nucleotide
acagkgtcgcatrrkkgrctayttkhcgcytycacctwttwsnagact

SEQ ID NO: 226 - DNA, 49 bp, Artificial sequence
  synthetic Family 946 Consensus
  misc_feature (4)..(4): n at position 4 can be G or no nucleotide
  misc_feature (5)..(5): n at position 5 can be C, G, T, or no nucleotide
  misc_feature (44)..(44): n at position 44 can be A, C, G, or no nucleotide
acanngtmgcatadtgggctdcwgrcgcmktcaaayctatttrnagact

SEQ ID NO: 227 - protein, 11 aa, Artificial sequence
  synthetic Membrane-targeting domain of Src-Flag-Vpx
MGSSKSKPKDP

SEQ ID NO: 228 - protein, 8 aa, Artificial sequence
  synthetic Viral protease cleavage domain
KARVLAEA

SEQ ID NO: 229 - protein, 458 aa, Homo sapiens
MTILGTTFGMVFSLLQVVSGESGYAQNGDLEDAELDDYSFSCYSQLEVNGSQHSLTCAFEDPDVNITNLEFEICGALVEVKCLNFRKLQEIYFIETKKFLLIGKSNICVKVGEKSLTCKKIDLTTIVKPEAPFDLSVVYREGANDFVVTFNTSHLQKKYVKVLMHDVAYRQEKDENKWTHVNLSSTKLTLLQRKLQPAAMYEIKVRSIPDHYFKGFWSEWSPSYYFRTPEINNSSGEMDPILLTISILSFFSVALLVILACVLWKKRIKPIVWPSLPDHKKTLEHLCKKPRKNLNVSFNPESFLDCQIHRVDDIQARDEVEGFLQDTFPQQLEESEKQRLGGDVQSPNCPSEDVVITPESFGRDSSLTCLAGNVSACDAPILSSSRSLDCRESGKNGPHVYQDLLLSLGTTNSTLPPPFSLQSGILTLNPVAQGQPILTSLGSNQEEAYVTMSSFYQN

SEQ ID NO: 230 - protein, 723 aa, Artificial sequence
  synthetic GFP - linker - P2A -IL7Ra IncPPCL codon(exceptP2A) and splice optimized
MSGGEELFAGIVPVLIELDGDVHGHKFSVRGEGEGDADYGKLEIKFICTTGKLPVPWPTLVTTLCYGIQCFARYPEHMKMNDFFKSAMPEGYIQERTIQFQDDGKYKTRGEVKFEGDTLVNRIELKGKDFKEDGNILGHKLEYSFNSHNVYIRPDKANNGLEANFKTRHNIEGGGVQLADHYQTNVPLGDGPVLIPINHYLSTQTKISKDRNEARDHMVLLESFSACCHTHGMDELYRGSGATNFSLLKQAGDVEENPGPMTILGTTFGMVFSLLQVVSGESGYAQNGDLEDAELDDYSFSCYSQLEVNGSQHSLTCAFEDPDVNITNLEFEICGALVEVKCLNFRKLQEIYFIETKKFLLIGKSNICVKVGEKSLTCKKIDLTTIVKPEAPFDLSVVYREGANDFVVTFNTSHLQKKYVKVLMHDVAYRQEKDENKWTHVNLSSTKLTLLQRKLQPAAMYEIKVRSIPDHYFKGFWSEWSPSYYFRTPEINNSSGEMDPILLPPCLTISILSFFSVALLVILACVLWKKRIKPIVWPSLPDHKKTLEHLCKKPRKNLNVSFNPESFLDCQIHRVDDIQARDEVEGFLQDTFPQQLEESEKQRLGGDVQSPNCPSEDVVITPESFGRDSSLTCLAGNVSACDAPILSSSRSLDCRESGKNGPHVYQDLLLSLGTTNSTLPPPFSLQSGILTLNPVAQGQPILTSLGSNQEEAYVTMSSFYQNQ

SEQ ID NO: 231 - protein, 733 aa, Artificial sequence
  synthetic GFP - linker - P2A - Myc Tag - IL7Ra IncPPCL codon(exceptP2A) and splice optimized
MSGGEELFAGIVPVLIELDGDVHGHKFSVRGEGEGDADYGKLEIKFICTTGKLPVPWPTLVTTLCYGIQCFARYPEHMKMNDFFKSAMPEGYIQERTIQFQDDGKYKTRGEVKFEGDTLVNRIELKGKDFKEDGNILGHKLEYSFNSHNVYIRPDKANNGLEANFKTRHNIEGGGVQLADHYQTNVPLGDGPVLIPINHYLSTQTKISKDRNEARDHMVLLESFSACCHTHGMDELYRGSGATNFSLLKQAGDVEENPGPMTILGTTFGMVFSLLQVVSGEQKLISEEDLESGYAQNGDLEDAELDDYSFSCYSQLEVNGSQHSLTCAFEDPDVNITNLEFEICGALVEVKCLNFRKLQEIYFIETKKFLLIGKSNICVKVGEKSLTCKKIDLTTIVKPEAPFDLSVVYREGANDFVVTFNTSHLQKKYVKVLMHDVAYRQEKDENKWTHVNLSSTKLTLLQRKLQPAAMYEIKVRSIPDHYFKGFWSEWSPSYYFRTPEINNSSGEMDPILLPPCLTISILSFFSVALLVILACVLWKKRIKPIVWPSLPDHKKTLEHLCKKPRKNLNVSFNPESFLDCQIHRVDDIQARDEVEGFLQDTFPQQLEESEKQRLGGDVQSPNCPSEDVVITPESFGRDSSLTCLAGNVSACDAPILSSSRSLDCRESGKNGPHVYQDLLLSLGTTNSTLPPPFSLQSGILTLNPVAQGQPILTSLGSNQEEAYVTMSSFYQNQ

SEQ ID NO: 232 - protein, 572 aa, Artificial sequence
  synthetic GFP - linker - P2A - IL7RaSP - Myc Tag - IL7RaIncPPCL C-terminal truncation codon(exceptP2A) and splice
MSGGEELFAGIVPVLIELDGDVHGHKFSVRGEGEGDADYGKLEIKFICTTGKLPVPWPTLVTTLCYGIQCFARYPEHMKMNDFFKSAMPEGYIQERTIQFQDDGKYKTRGEVKFEGDTLVNRIELKGKDFKEDGNILGHKLEYSFNSHNVYIRPDKANNGLEANFKTRHNIEGGGVQLADHYQTNVPLGDGPVLIPINHYLSTQTKISKDRNEARDHMVLLESFSACCHTHGMDELYRGSGATNFSLLKQAGDVEENPGPMTILGTTFGMVFSLLQVVSGEQKLISEEDLESGYAQNGDLEDAELDDYSFSCYSQLEVNGSQHSLTCAFEDPDVNITNLEFEICGALVEVKCLNFRKLQEIYFIETKKFLLIGKSNICVKVGEKSLTCKKIDLTTIVKPEAPFDLSVVYREGANDFVVTFNTSHLQKKYVKVLMHDVAYRQEKDENKWTHVNLSSTKLTLLQRKLQPAAMYEIKVRSIPDHYFKGFWSEWSPSYYFRTPEINNSSGEMDPILLPPCLTISILSFFSVALLVILACVLWKKRIKPIVWPSLPDHKKTLEHLCKKPRKVSVFGA

SEQ ID NO: 233 - protein, 562 aa, Artificial sequence
  synthetic GFP - linker - P2A - IL7RaSP - IL7RaIncPPCL C-terminal truncation codon(exceptP2A) and splice optimized
MSGGEELFAGIVPVLIELDGDVHGHKFSVRGEGEGDADYGKLEIKFICTTGKLPVPWPTLVTTLCYGIQCFARYPEHMKMNDFFKSAMPEGYIQERTIQFQDDGKYKTRGEVKFEGDTLVNRIELKGKDFKEDGNILGHKLEYSFNSHNVYIRPDKANNGLEANFKTRHNIEGGGVQLADHYQTNVPLGDGPVLIPINHYLSTQTKISKDRNEARDHMVLLESFSACCHTHGMDELYRGSGATNFSLLKQAGDVEENPGPMTILGTTFGMVFSLLQVVSGESGYAQNGDLEDAELDDYSFSCYSQLEVNGSQHSLTCAFEDPDVNITNLEFEICGALVEVKCLNFRKLQEIYFIETKKFLLIGKSNICVKVGEKSLTCKKIDLTTIVKPEAPFDLSVVYREGANDFVVTFNTSHLQKKYVKVLMHDVAYRQEKDENKWTHVNLSSTKLTLLQRKLQPAAMYEIKVRSIPDHYFKGFWSEWSPSYYFRTPEINNSSGEMDPILLPPCLTISILSFFSVALLVILACVLWKKRIKPIVWPSLPDHKKTLEHLCKKPRKVSVFGA

SEQ ID NO: 234 - protein, 824 aa, Artificial sequence
  synthetic GFP - linker - P2A - eTag -  IL7RaIncPPCL N-terminal deletion codon(exceptP2A) and splice optimized
MSGGEELFAGIVPVLIELDGDVHGHKFSVRGEGEGDADYGKLEIKFICTTGKLPVPWPTLVTTLCYGIQCFARYPEHMKMNDFFKSAMPEGYIQERTIQFQDDGKYKTRGEVKFEGDTLVNRIELKGKDFKEDGNILGHKLEYSFNSHNVYIRPDKANNGLEANFKTRHNIEGGGVQLADHYQTNVPLGDGPVLIPINHYLSTQTKISKDRNEARDHMVLLESFSACCHTHGMDELYRGSGATNFSLLKQAGDVEENPGPMLLLVTSLLLCELPHPAFLLIPRKVCNGIGIGEFKDSLSINATNIKHFKNCTSISGDLHILPVAFRGDSFTHTPPLDPQELDILKTVKEITGFLLIQAWPENRTDLHAFENLEIIRGRTKQHGQFSLAVVSLNITSLGLRSLKEISDGDVIISGNKNLCYANTINWKKLFGTSGQKTKIISNRGENSCKATGQVCHALCSPEGCWGPEPRDCVSCRNVSRGRECVDKCNLLEGEPREFVENSECIQCHPECLPQAMNITCTGRGPDNCIQCAHYIDGPHCVKTCPAGVMGENNTLVWKYADAGHVCHLCHPNCTYGCTGPGLEGCPTNGPEINNSSGEMDPILLPPCLTISILSFFSVALLVILACVLWKKRIKPIVWPSLPDHKKTLEHLCKKPRKNLNVSFNPESFLDCQIHRVDDIQARDEVEGFLQDTFPQQLEESEKQRLGGDVQSPNCPSEDVVITPESFGRDSSLTCLAGNVSACDAPILSSSRSLDCRESGKNGPHVYQDLLLSLGTTNSTLPPPFSLQSGILTLNPVAQGQPILTSLGSNQEEAYVTMSSFYQNQ

SEQ ID NO: 235 - protein, 593 aa, Artificial sequence
  synthetic MV(ed)-HD24
MNREHLMIDRPYVLLAVLFVMSLSLIGLLAIAGIRLHRAAIYTAEIHKSLSTNLDVTNSIEHQVKDVLTPLFKIIGDEVGLRTPQRFTDLVKFISDKIKFLNPDREYDFRDLTWCINPPERIKLDYDQYCADVAAEELMNALVNSTLLETRTTNQFLAVSKGNCSGPTTIRGQFSNMSLSLLDLYLSRGYNVSSIVTMTSQGMYGGTYLVEKPNLSSKRSELSQLSMYRVFEVGVIRNPGLGAPVFHMTNYLEQPVSNDLSNCMVALGELKLAALCHGEDSITIPYQGSGKGVSFQLVKLGVWKSPTDMQSWVPLSTDDPVIDRLYLSSHRGVIADNQAKWAVPTTRTDDKLRMETCFQQACKGKIQALCENPEWAPLKDNRIPSYGVLSVDLSLTVELKIKIASGFGPLITHGSGMDLYKSNHNNVYWLTIPPMKNLALGVINTLEWIPRFKVSPNLFTVPIKEAGEDCHAPTYLPAEVDGDVKLSSNLVILPGQDLQYVLATYDTSRVEHAVVYYVYSPGRSFSYFYPFRLPIKGVPIELQVECFTWDQKLWCRHFCVLADSESGGHITHSGMVGMGVSCTVTREDGTNRR

SEQ ID NO: 236 - DNA, 1275 bp, Mesoplasma florum
aaaaaaaataaaatcaatagcaaatattaagatttttaagaaataaaaaattaatattaatttacaactgaatataaaagaaacttatacagggtagcataatgggctactgaccccgccttcaaacctatttggagactataagtgaaaaaccactctttaattattaaagtttctttttatgtccaaaagacaagaagaaacttttttatttagttgaatttataataagagaaaaagaaaggatattatatggcaaaaataaaaaaccaatattacaacgagtctgtttcgccaattgaatatgcgcaacaaggatttaaaggaaaaatgcgttcagtaaactgaaacgtagtaaatgatgaaaaagatttagaggtatgaaatagaattacacaaaacttctgattgcctgaaaaaattccagtttcaaatgatttaacttcatgaagaactttgacaccagaatgacaagaattaattacaagaacttttacaggattaacattgttagatacaattcaagctactgttggtgatgtggctcaagttcctaactcattaactgaccatgaacaagtaatttacacaaactttgcatttatggttgcagttcacgctagatcatatggttcaatcttttcaactttatgttcaagtgaacaaattgaagaggctcatgaatgagttatcaatacagaaacattacaagaaagagctaaagcattaattccttattatgtgaatgatgaccctttaaagtcaaaagttgcagctgctttaatgccaggcttcttattatatggaggcttctatttaccattttacctatcagctagaggtaaattaccaaacacttcagatattattagattaatattaagagataaagttatacataactactatagtggttataaatatcaaaagaaagttgctaaactttctccagaaaaacaagctgaaatgaaagaatttgtttttaaattattatatgaattaatagatttagaaaaagcttatttgaaagaattgtatgaggattttggattagctgatgatgctattagatttagtgtttacaacgcaggtaaatttttacaaaatttaggttatgattcaccgtttacagaagaagaaacaagaattgagccagaaatattcacacaattatcagctagagctgatgaaaaccatgatttcttttcagggaatggctcatcatatattatgggagtttcagaagaaactgaagatgacgattgggagttttaa

SEQ ID NO: 237 - RNA, 64 nt, Mesoplasma florum
acuuauacaggguagcauaaugggcuacugaccccgccuucaaaccuauuuggagacuauaagu

SEQ ID NO: 238 - RNA, 69 nt, Artificial sequence
  synthetic Deoxyguanosine riboswitch aptamer mutations
  misc_feature (10)..(13): n at positions 10-13 can be A, C, G, or T
  misc_feature (27)..(29): n at positions 27-29 can be A, C, G, or T
  misc_feature (31)..(32): n at positions 31-32 can be A, C, G, or T
  misc_feature (33)..(40): n at positions 33-40 can be A, C, G, T, or no nucleotide
  misc_feature (44)..(46): n at positions 44-46 can be A, C, G, or T
  misc_feature (57)..(59): n at positions 57-59 can be A, C, G, or T
acuuauacannnnagcauaaugggcunnngnnnnnnnnnngccnnnaaaccuauuunnngacuauaagu

SEQ ID NO: 239 - DNA, 84 bp, Artificial sequence
  synthetic Oligo library for screen
  misc_feature (19)..(21): n at positions 19-21 can be A, C, G, or T
  misc_feature (32)..(34): n at positions 32-34 can be A, C, G, or T
  misc_feature (38)..(39): n at positions 38-39 can be A, C, G, or T
  misc_feature (40)..(47): n at positions 40-47 can be A, C, G, T, or no nucleotide
  misc_feature (49)..(51): n at positions 49-51 can be A, C, G, or T
  misc_feature (65)..(68): n at positions 65-68 can be A, C, G, or T
cgcgcgacacttatagtcnnnaaataggtttnnnggcnnnnnnnnnncnnnagcccattatgctnnnntgtataagtgccgccc

SEQ ID NO: 240 - DNA, 33 bp, Artificial sequence
  synthetic T7 promoter amplification primer
taatacgactcactatagggcggcacttataca

SEQ ID NO: 241 - DNA, 18 bp, Artificial sequence
  synthetic Reverse amplification primer
cgcgcgacacttatagtc

SEQ ID NO: 242 - DNA, 915 bp, Bacillus subtilis
tcaaaagcctggcggcgcggtcgtcagactcttttatatcgaatccccttgaaatacgaatgatatctaaaaaaacaaaattaaagttcgggaatttttattttcagcctatgcaagagattagaatcttgatataatttattacaatataataggaacactcatataatcgcgtggatatggcacgcaagtttctaccgggcaccgtaaatgtccgactatgggtgagcaatggaaccgcacgtgtacggttttttgtgatatcagcattgcttgctctttatttgagcgggcaatgctttttttattctcataacggaggtagacaggatggaagcactgaaacggaaaatagaggaagaaggcgtcgtattatctgatcaggtattgaaagtggattcttttttgaatcaccaaattgatccgctgcttatgcagagaattggtgatgaatttgcgtctaggtttgcaaaagacggtattaccaaaattgtgacaatcgaatcatcaggtatcgctcccgctgtaatgacgggcttgaagctgggtgtgccagttgtcttcgcgagaaagcataaatcgttaacactcaccgacaacttgctgacagcgtctgtttattcctttacgaagcaaacagaaagccaaatcgcagtgtctgggacccacctgtcggatcaggatcatgtgctgattatcgatgattttttggcaaatggacaggcagcgcacgggcttgtgtcgattgtgaagcaagcgggagcttctattgcgggaatcggcattgttattgaaaagtcatttcagccgggaagagatgaacttgtaaaactgggctaccgagtggaatctttggcaagaattcagtctttagaagaaggaaaagtgtccttcgtacaggaggttcattcatga

SEQ ID NO: 243 - RNA, 69 nt, Bacillus subtilis
cacucauauaaucgcguggauauggcacgcaaguuucuaccgggcaccguaaauguccgacuaugggug

SEQ ID NO: 244 - RNA, 74 nt, Artificial sequence
  synthetic Guanosine xpt riboswitch aptamer mutations
  misc_feature (11)..(14): n at positions 11-14 can be A, C, G, or T
  misc_feature (30)..(35): n at positions 30-35 can be A, C, G, or T
  misc_feature (36)..(43): n at positions 36-43 can be A, C, G, T, or no nucleotide
  misc_feature (47)..(49): n at positions 47-49 can be A, C, G, or T
  misc_feature (61)..(63): n at positions 61-63 can be A, C, G, or T
cacucauauannnncguggauauggcacgnnngnnnnnnnnnnaccnnnuaccguaaaugnnngacuaugggug

SEQ ID NO: 245 - DNA, 89 bp, Artificial sequence
  synthetic Oligo library for screen
  misc_feature (20)..(22): n at positions 20-22 can be A, C, G, or T
  misc_feature (34)..(36): n at positions 34-36 can be A, C, G, or T
  misc_feature (40)..(41): n at positions 40-41 can be A, C, G, or T
  misc_feature (42)..(49): n at positions 42-49 can be A, C, G, T, or no nucleotide
  misc_feature (51)..(53): n at positions 51-53 can be A, C, G, or T
  misc_feature (69)..(72): n at positions 69-72 can be A, C, G, or T
cgcgcgaccacccatagtcnnncatttacggtgnnnggtnnnnnnnnnncnnncgtgccatatccacgnnnntatatgagtggccgccc

SEQ ID NO: 246 - DNA, 34 bp, Artificial sequence
  synthetic T7 promoter amplification primer
taatacgactcactatagggcggccactcatata

SEQ ID NO: 247 - DNA, 19 bp, Artificial sequence
  synthetic Reverse amplification primer
cgcgcgaccacccatagtc

SEQ ID NO: 248 - RNA, 152 nt, Artificial sequence
  synthetic Oligo 1 Transcribed RNA
gggcggcacuuauacaggguagcauaaugggcuacugacgccuucaaaccuauuuggagacuauaagugucgcgcggggcggcacuuauacaggguagcauaaugggcuacugacgccuucaaaccuauuuggagacuauaagugucgcgcg

SEQ ID NO: 249 - DNA, 76 bp, Artificial sequence
  synthetic Oligo 1 Synthesized template
cgcgcgacacttatagtctccaaataggtttgaaggcgtcagtagcccattatgctaccctgtataagtgccgccc

SEQ ID NO: 250 - RNA, 79 nt, Artificial sequence
  synthetic Oligo 2 Transcribed RNA
gggcggcacuuauacaggguagcauaaugggcuacugaccccgccuucaaaccuauuuggagacuauaagugucgcgcg

SEQ ID NO: 251 - DNA, 79 bp, Artificial sequence
  synthetic Oligo 2 Synthesized template
cgcgcgacacttatagtctccaaataggtttgaaggcggggtcagtagcccattatgctaccctgtataagtgccgccc

SEQ ID NO: 252 - protein, 560 aa, Artificial sequence
  synthetic DAFss-aCD3scFv(UCHT1)IgG1 Fc-CD14GPI
MTVARPSVPAALPLLGELPRLLLLVLLCLPDIQMTQSPSSLSASVGDRVTITCRASQDIRNYLNWYQQKPGKAPKLLIYYTSRLESGVPSRFSGSGSGTDYTLTISSLQPEDFATYYCQQGNTLPWTFGQGTKVEIKGGGGSGGGGSGGGGSEVQLVESGGGLVQPGGSLRLSCAASGYSFTGYTMNWVRQAPGKGLEWVALINPYKGVSTYNQKFKDRFTISVDKSKNTAYLQMNSLRAEDTAVYYCARSGYYGDSDWYFDVWGQGTLVTVSSEPKSCDKTHTCPPCPAPELLGGPSVFLFPPKPKDTLMISRTPEVTCVVVDVSHEDPEVKFNWYVDGVEVHNAKTKPREEQYNSTYRVVSVLTVLHQDWLNGKEYKCKVSNKALPAPIEKTISKAKGQPREPQVYTLPPSREEMTKNQVSLTCLVKGFYPSDIAVEWESNGQPENNYKTTPPVLDSDGSFFLYSKLTVDKSRWQQGNVFSCSVMHEALHNHYTQKSLSLSPGVDNLTLDGNPFLVPGTALPHEGSMNSGVVPACARSTLSVGVSGTLVLLQGARGFA

SEQ ID NO: 253 - protein, 276 aa, Artificial sequence
  synthetic DAFss-CD80ECD-CD16GPI
MTVARPSVPAALPLLGELPRLLLLVLLCLPVIHVTKEVKEVATLSCGHNVSVEELAQTRIYWQKEKKMVLTMMSGDMNIWPEYKNRTIFDITNNLSIVILALRPSDEGTYECVVLKYEKDAFKREHLAEVTLSVKADFPTPSISDFEIPTSNIRRIICSTSGGFPEPHLSWLENGEELNAINTTVSQDPETELYAVSSKLDFNMTTNHSFMCLIKYGHLRVNQTFNWNTTKQEHFPDNVSTISSFSPPGYQVSFCLVMVLLFAVDTGLYFSVKTNI

SEQ ID NO: 254 - protein, 533 aa, Artificial sequence
  synthetic DAFss-IL7-DAF
MATTMTVARPSVPAALPLLGELPRLLLLVLLCLPADCDIEGKDGKQYESVLMVSIDQLLDSMKEIGSNCLNNEFNFFKRHICDANKEGMFLFRAARKLRQFLKMNSTGDFDLHLLKVSEGTTILLNCTGQVKGRKPAALGEAQPTKSLEENKSLKEQKKLNDLCFLKRLLQEIKTCWNKILMGTKEHCGLPPDVPNAQPALEGRTSFPEDTVITYKCEESFVKIPGEKDSVICLKGSQWSDIEEFCNRSCEVPTRLNSASLKQPYITQNYFPVGTVVEYECRPGYRREPSLSPKLTCLQNLKWSTAVEFCKKKSCPNPGEIRNGQIDVPGGILFGATISFSCNTGYKLFGSTSSFCLISGSSVQWSDPLPECREIYCPAPPQIDNGIIQGERDHYGYRQSVTYACNKGFTMIGEHSIYCTVNNDEGEWSGPPPECRGKSLTSKVPPTVQKPTTVNVPTTEVSPTSQKTTTKTTTPNAQATRSTPVSRTTKHFHETTPNKGSGTTSGTTRLLSGHTCFTLTGLLGTLVTMGLLT

SEQ ID NO: 255 - DNA, 1823 bp, Artificial sequence
  synthetic EF-1a promoter with miRs
ggctccggtgcccgtcagtgggcagagcgcacatcgcccacagtccccgagaagttggggggaggggtcggcaattgaaccggtgcctagagaaggtggcgcggggtaaactgggaaagtgatgtcgtgtactggctccgcctttttcccgagggtgggggagaaccgtatataagtgcagtagtcgccgtgaacgttctttttcgcaacgggtttgccgccagaacacaggtaagtgccgtgtgtggttcccgcgggcctggcctctttacgggttatggcccttgcgtgccttgaattacttccacctggctgcagtacgtgattcttgatcccgagcttcgggttggaagtgggtgggagagttcgaggccttgcgcttaaggagccccttcgcctcgtgcttgagttgaggcctggcctgggcgctggggccgccgcgtgcgaatctggtggcaccttcgcgcctgtctcgctgctttcgataagtctctagccatttaaaatttttgatgacctgctgcgacgctttttttctggcaagatagtcttgtaaatgcgggccaagatctgcacactggtatttcggtttttggggccgcgggcggcgacggggcccgtgcgtcccagcgcacatgttcggcgaggcggggcctgcgagcgcggccaccgagaatcggacgggggtagtctcaagctggccggcctgctctggtgcctggcctcgcgccgccgtgtatcgccccgccctgggcggcaaggctggcccggtcggcaccagttgcgtgagcggaaagatggccgcttcccggccctgctgcagggagctcaaaatggaggacgcggcgctcgggagagcgggcgggtgagtcacccacacaaaggaaaagggcctttccgtcctcagccgtcgcttcatgtgactccactgagtaccgggcgccgtccaggcacctcgattagttcctggaggcttgctgaaggctgtatgctgacatggtacagttcaatggtggttttggccactgactgaccaccattgctgtaccatgtcaggacacaaggcctgttactagcactcacatggaacaaatggcccacattggtgccggatgaagctcttatgttgcacggtcatctggaggcttgctgaaggctgtatgctgtcagtctgttcatcttctggcgttttggccactgactgacgccagaaggaacagactgacaggacacaaggcctgttactagcactcacatggaacaaatggccgttgccggagtcttggcagcgagagatcactatcaactaactggaggcttgctgaaggctgtatgctgaagcgtgaagtgaatcaacgggttttggccactgactgacccgttgatacttcacgcttcaggacacaaggcctgttactagcactcacatggaacaaatggccgtgttaattgtccatgtagcgaggcatccttatggcgtggctggaggcttgctgaaggctgtatgctggcagtatcctagtacattgacgttttggccactgactgacgtcaatgttaggatactgccaggacacaaggcctgttactagcactcacatggaacaaatggccgcttttggagtacgtcgtctttaggttggggggaggggttttatgcgatggagtttccccacactgagtgggtggagactgaagttaggccagcttggcacttgatgtaattctccttggaatttgccctttttgagtttggatcttggttcattctcaagcctcagacagtggttcaaagtttttttcttccatttcaggtgtcgtga

SEQ ID NO: 256 - DNA, 28 bp, Mus musculus
ctggaggcttgctgaaggctgtatgctg

SEQ ID NO: 257 - DNA, 21 bp, Artificial sequence
  Synthetic DNA encoding MiRNA stem
acatggtacagttcaatggtg

SEQ ID NO: 258 - DNA, 19 bp, Artificial sequence
  synthetic DNA encoding loop
gttttggccactgactgac

SEQ ID NO: 259 - DNA, 19 bp, Artificial sequence
  synthetic DNA encoding stem
caccattgctgtaccatgt

SEQ ID NO: 260 - DNA, 45 bp, Mus musculus
caggacacaaggcctgttactagcactcacatggaacaaatggcc

SEQ ID NO: 261 - DNA, 21 bp, Artificial sequence
  Synthetic DNA encoding MiRNA stem
tcagtctgttcatcttctggc

SEQ ID NO: 262 - DNA, 19 bp, Artificial sequence
  Synthetic DNA encoding MiRNA stem
gccagaaggaacagactga

SEQ ID NO: 263 - DNA, 21 bp, Artificial sequence
  Synthetic DNA encoding MiRNA stem
aagcgtgaagtgaatcaacgg

SEQ ID NO: 264 - DNA, 19 bp, Artificial sequence
  Synthetic DNA encoding MiRNA stem
ccgttgatacttcacgctt

SEQ ID NO: 265 - DNA, 21 bp, Artificial sequence
  Synthetic DNA encoding MiRNA stem
gcagtatcctagtacattgac

SEQ ID NO: 266 - DNA, 19 bp, Artificial sequence
  Synthetic DNA encoding MiRNA stem
gtcaatgttaggatactgc

SEQ ID NO: 267 - DNA, 21 bp, Artificial sequence
  Synthetic DNA encoding MiRNA stem
atatgtacttggctggacagc

SEQ ID NO: 268 - DNA, 19 bp, Artificial sequence
  Synthetic DNA encoding MiRNA stem
gctgtccacaagtacatat

SEQ ID NO: 269 - DNA, 39 bp, Artificial sequence
  synthetic DNA encoding linker
cacattggtgccggatgaagctcttatgttgccggtcat

SEQ ID NO: 270 - DNA, 21 bp, Artificial sequence
  Synthetic DNA encoding MiRNA stem
ctgttaatgctaatcgtgata

SEQ ID NO: 271 - DNA, 18 bp, Artificial sequence
  Synthetic DNA encoding MiRNA stem
tatcacgattattaacag

SEQ ID NO: 272 - DNA, 40 bp, Artificial sequence
  synthetic DNA encoding linker
gttgccggagtcttggcagcgagagatcactatcaactaa

SEQ ID NO: 273 - DNA, 21 bp, Artificial sequence
  Synthetic DNA encoding MiRNA stem
taccagtttagcacgaagctc

SEQ ID NO: 274 - DNA, 19 bp, Artificial sequence
  Synthetic DNA encoding MiRNA stem
gagcttcgctaaactggta

SEQ ID NO: 275 - DNA, 40 bp, Artificial sequence
  synthetic DNA encoding linker
gtgttaattgtccatgtagcgaggcatccttatggcgtgg

SEQ ID NO: 276 - DNA, 21 bp, Artificial sequence
  Synthetic DNA encoding MiRNA stem
tgccgctgaaatccaaggcaa

SEQ ID NO: 277 - DNA, 19 bp, Artificial sequence
  Synthetic DNA encoding MiRNA stem
ttgccttgtttcagcggca

SEQ ID NO: 278 - protein, 534 aa, Artificial sequence
  Synthetic UCHT1scFvFc-GPI
MDMRVPAQLLGLLLLWLSGARCDIQMTQSPSSLSASVGDRVTITCRASQDIRNYLNWYQQKPGKAPKLLIYYTSRLESGVPSRFSGSGSGTDYTLTISSLQPEDFATYYCQQGNTLPWTFGQGTKVEIKGGGGSGGGGSGGGGSEVQLVESGGGLVQPGGSLRLSCAASGYSFTGYTMNWVRQAPGKGLEWVALINPYKGVSTYNQKFKDRFTISVDKSKNTAYLQMNSLRAEDTAVYYCARSGYYGDSDWYFDVWGQGTLVTVSSEPKSCDKTHTCPPCPAPELLGGPSVFLFPPKPKDTLMISRTPEVTCVVVDVSHEDPEVKFNWYVDGVEVHNAKTKPREEQYNSTYRVVSVLTVLHQDWLNGKEYKCKVSNKALPTPIEKTISKAKGQPREPQVYTLPPSREEMTKNQVSLTCLVKGFYPSDIAVEWESNGQPENNYKTTPPVLDSDGSFFLYSKLTVDKSRWQQGNVFSCSVMHEALHNHYTQKSLSLSPGPNKGSGTTSGTTRLLSGHTCFTLTGLLGTLVTMGLLT

SEQ ID NO: 279 - protein, 530 aa, Artificial sequence
  Synthetic OKT3scFvFc-GPI
MDMRVPAQLLGLLLLWLSGARCQIVLTQSPAIMSASPGEKVTMTCSASSSVSYMNWYQQKSGTSPKRWIYDTSKLASGVPAHFRGSGSGTSYSLTISGMEAEDAATYYCQQWSSNPFTFGSGTKLEINGGGGSGGGGSGGGGSQVQLQQSGAELARPGASVKMSCKASGYTFTRYTMHWVKQRPGQGLEWIGYINPSRGYTNYNQKFKDKATLTTDKSSSTAYMQLSSLTSEDSAVYYCARYYDDHYCLDYWGQGTTLTVSSEPKSCDKTHTCPPCPAPELLGGPSVFLFPPKPKDTLMISRTPEVTCVVVDVSHEDPEVKFNWYVDGVEVHNAKTKPREEQYNSTYRVVSVLTVLHQDWLNGKEYKCKVSNKALPAPIEKTISKAKGQPREPQVYTLPPSREEMTKNQVSLTCLVKGFYPSDIAVEWESNGQPENNYKTTPPVLDSDGSFFLYSKLTVDKSRWQQGNVFSCSVMHEALHNHYTQKSLSLSPGPNKGSGTTSGTTRLLSGHTCFTLTGLLGTLVTMGLLT

SEQ ID NO: 280 - protein, 280 aa, Artificial sequence
  Synthetic hCD80-CD16 GPI
MGHTRRQGTSPSKCPYLNFFQLLVLAGLSHFCSGVIHVTKEVKEVATLSCGHNVSVEELAQTRIYWQKEKKMVLTMMSGDMNIWPEYKNRTIFDITNNLSIVILALRPSDEGTYECVVLKYEKDAFKREHLAEVTLSVKADFPTPSISDFEIPTSNIRRIICSTSGGFPEPHLSWLENGEELNAINTTVSQDPETELYAVSSKLDFNMTTNHSFMCLIKYGHLRVNQTFNWNTTKQEHFPDNVSTISSFSPPGYQVSFCLVMVLLFAVDTGLYFSVKTNI

SEQ ID NO: 281 - protein, 120 aa, Artificial sequence
  Synthetic Target 1 MRB VH
EVQLVQSGAEVKKPGATVKISCKVSGYSFWGATMNWIRQPPGKGLEWIGLIKPSNGGTSYNQKFKGRVTISADKSISTAYLQWSSLKASDTAMYYCAHGHYESYEAMDYWGQGTLVTVSS

SEQ ID NO: 282 - protein, 107 aa, Artificial sequence
  Synthetic Target 1 MRB VL
DIQMTQSPSSLSASVGDRVTITCKASQDVVSAVAWYQQKPGQAPRLLIYWQDTRHTGVPSRFSGSGSGTEFTLTISSLQPDDFATYYCQEHFSPPLTFGQGTKVEIK

SEQ ID NO: 283 - protein, 15 aa, Artificial sequence
  Synthetic Linker 1
GGGGSGGGGSGGGGS

SEQ ID NO: 284 - protein, 357 aa, Artificial sequence; identical to SEQ ID NO: 78
  Synthetic C1 control polypeptide containing GMCSF alpha chain signal sequence (amino acids 1-22) and eTAG (amino acids 23-357)

SEQ ID NO: 285 - protein, 240 aa, Artificial sequence
  Synthetic OKT3 ScFv
QIVLTQSPAIMSASPGEKVTMTCSASSSVSYMNWYQQKSGTSPKRWIYDTSKLASGVPAHFRGSGSGTSYSLTISGMEAEDAATYYCQQWSSNPFTFGSGTKLEINGGGGSGGGGSGGGGSQVQLQQSGAELARPGASVKMSCKASGYTFTRYTMHWVKQRPGQGLEWIGYINPSRGYTNYNQKFKDKATLTTDKSSSTAYMQLSSLTSEDSAVYYCARYYDDHYCLDYWGQGTTLTVSS

SEQ ID NO: 286 - protein, 532 aa, Artificial sequence
  Synthetic DAFss-IL7-DAF fusion
MTVARPSVPAALPLLGELPRLLLLVLLCLPAVWGDCDIEGKDGKQYESVLMVSIDQLLDSMKEIGSNCLNNEFNFFKRHICDANKEGMFLFRAARKLRQFLKMNSTGDFDLHLLKVSEGTTILLNCTGQVKGRKPAALGEAQPTKSLEENKSLKEQKKLNDLCFLKRLLQEIKTCWNKILMGTKEHCGLPPDVPNAQPALEGRTSFPEDTVITYKCEESFVKIPGEKDSVICLKGSQWSDIEEFCNRSCEVPTRLNSASLKQPYITQNYFPVGTVVEYECRPGYRREPSLSPKLTCLQNLKWSTAVEFCKKKSCPNPGEIRNGQIDVPGGILFGATISFSCNTGYKLFGSTSSFCLISGSSVQWSDPLPECREIYCPAPPQIDNGIIQGERDHYGYRQSVTYACNKGFTMIGEHSIYCTVNNDEGEWSGPPPECRGKSLTSKVPPTVQKPTTVNVPTTEVSPTSQKTTTKTTTPNAQATRSTPVSRTTKHFHETTPNKGSGTTSGTTRLLSGHTCFTLTGLLGTLVTMGLLT

SEQ ID NO: 287 - protein, 564 aa, Artificial sequence
  Synthetic DAFss-aCD3scFv(UCHT1)IgG1 Fc-CD14GPI
MTVARPSVPAALPLLGELPRLLLLVLLCLPAVWGDIQMTQSPSSLSASVGDRVTITCRASQDIRNYLNWYQQKPGKAPKLLIYYTSRLESGVPSRFSGSGSGTDYTLTISSLQPEDFATYYCQQGNTLPWTFGQGTKVEIKGGGGSGGGGSGGGGSEVQLVESGGGLVQPGGSLRLSCAASGYSFTGYTMNWVRQAPGKGLEWVALINPYKGVSTYNQKFKDRFTISVDKSKNTAYLQMNSLRAEDTAVYYCARSGYYGDSDWYFDVWGQGTLVTVSSEPKSCDKTHTCPPCPAPELLGGPSVFLFPPKPKDTLMISRTPEVTCVVVDVSHEDPEVKFNWYVDGVEVHNAKTKPREEQYNSTYRVVSVLTVLHQDWLNGKEYKCKVSNKALPAPIEKTISKAKGQPREPQVYTLPPSREEMTKNQVSLTCLVKGFYPSDIAVEWESNGQPENNYKTTPPVLDSDGSFFLYSKLTVDKSRWQQGNVFSCSVMHEALHNHYTQKSLSLSPGVDNLTLDGNPFLVPGTALPHEGSMNSGVVPACARSTLSVGVSGTLVLLQGARGFA

SEQ ID NO: 288 - protein, 280 aa, Artificial sequence
  Synthetic DAFss-CD80ECD-CD16GPI
MTVARPSVPAALPLLGELPRLLLLVLLCLPAVWGVIHVTKEVKEVATLSCGHNVSVEELAQTRIYWQKEKKMVLTMMSGDMNIWPEYKNRTIFDITNNLSIVILALRPSDEGTYECVVLKYEKDAFKREHLAEVTLSVKADFPTPSISDFEIPTSNIRRIICSTSGGFPEPHLSWLENGEELNAINTTVSQDPETELYAVSSKLDFNMTTNHSFMCLIKYGHLRVNQTFNWNTTKQEHFPDNVSTISSFSPPGYQVSFCLVMVLLFAVDTGLYFSVKTNI

SEQ ID NO: 289 - protein, 119 aa, Artificial sequence
  Synthetic Target 2 MRB VH
QVQLQESGPGLVKPSQTLSLTCTVSGYSITTGEYWNWVRQARGQRLEWIGYITYDGSKNYNPSLKNRVTISVDTSKNQFSLKLSSVTAADTAVYYCSRFEGVWYGLDYWGQGTLVTVSS

SEQ ID NO: 290 - protein, 111 aa, Artificial sequence
  Synthetic Target 2 MRB VL
AIQLTQSPSSLSASVGDRVTITCRASESVDRYGNSFIHWYQQKPGKAPKLLIYRTYNLESGIPARFSGSGSGTEFTLTISSLQSEDFAVYYCQQTNEDPWTFGQGTKVEIK

SEQ ID NO: 291 - protein, 30 aa, Artificial sequence; identical to SEQ ID NO: 54
  Synthetic Linker2